European Patent Specification EP 4 211 228 B1, published November 5, 2025. Title: T CELL PHENOTYPES ASSOCIATED WITH RESPONSE TO ADOPTIVE CELL THERAPY. Applicant: THE UNITED STATES OF AMERICA, AS REPRESENTED BY THE SECRETARY, DEPARTMENT OF HEALTH AND HUMAN SERVICES. The sequence listing filed with the application follows.

SEQUENCE LISTING (19 sequences)

SEQ ID NO: 1 - DNA, 12493 bp, Homo sapiens
acggagacggaccacagcaagcagaggctgggggggggaaagacgaggaaagaggaggaaaacaaaagctgctacttatggaagatacaaaggagtctaacgtgaagacattttgctccaagaatatcctagccatccttggcttctcctctatcatagctgtgatagctttgcttgctgtggggttgacccagaacaaagcattgccagaaaacgttaagtatgggattgtgctggatgcgggttcttctcacacaagtttatacatctataagtggccagcagaaaaggagaatgacacaggcgtggtgcatcaagtagaagaatgcagggttaaaggtcctggaatctcaaaatttgttcagaaagtaaatgaaataggcatttacctgactgattgcatggaaagagctagggaagtgattccaaggtcccagcaccaagagacacccgtttacctgggagccacggcaggcatgcggttgctcaggatggaaagtgaagagttggcagacagggttctggatgtggtggagaggagcctcagcaactacccctttgacttccagggtgccaggatcattactggccaagaggaaggtgcctatggctggattactatcaactatctgctgggcaaattcagtcagaaaacaaggtggttcagcatagtcccatatgaaaccaataatcaggaaacctttggagctttggaccttgggggagcctctacacaagtcacttttgtaccccaaaaccagactatcgagtccccagataatgctctgcaatttcgcctctatggcaaggactacaatgtctacacacatagcttcttgtgctatgggaaggatcaggcactctggcagaaactggccaaggacattcaggttgcaagtaatgaaattctcagggacccatgctttcatcctggatataagaaggtagtgaacgtaagtgacctttacaagaccccctgcaccaagagatttgagatgactcttccattccagcagtttgaaatccagggtattggaaactatcaacaatgccatcaaagcatcctggagctcttcaacaccagttactgcccttactcccagtgtgccttcaatgggattttcttgccaccactccagggggattttggggcattttcagctttttactttgtgatgaagtttttaaacttgacatcagagaaagtctctcaggaaaaggtgactgagatgatgaaaaagttctgtgctcagccttgggaggagataaaaacatcttacgctggagtaaaggagaagtacctgagtgaatactgcttttctggtacctacattctctccctccttctgcaaggctatcatttcacagctgattcctgggagcacatccatttcattggcaagatccagggcagcgacgccggctggactttgggctacatgctgaacctgaccaacatgatcccagctgagcaaccattgtccacacctctctcccactccacctatgtcttcctcatggttctattctccctggtccttttcacagtggccatcataggcttgcttatctttcacaagccttcatatttctggaaagatatggtatagcaaaagcagctgaaatatgctggctggagtgaggaaaaaaatcgtccagggagcattttcctccatcgcagtgttcaaggccatccttccctgtctgccagggccagtcttgacgagtgtgaagcttccttggcttttactgaagcctttcttttggaggtattcaatatcctttgcctcaaggacttcggcagatactgtctctttcatgagtttttcccagctacacctttctcctttgtactttgtgcttgtataggttttaaagacctgacacctttcataatctttgctttataaaagaacaatattgactttgtctagaagaactgagagtcttgagtcctgtgataggaggctgagctggctgaaagaagaatctcaggaactggttcagttgtactctttaagaacccctttctctctcctgtttgccatccattaagaaagccatatgatgcctttggagaaggcagacacacattccattcccagcctgctctgtgggtaggagaattttctacagtaggcaaatatgtgctaaagccaaagagttttataaggaaatatatgtgctcatgcagtcaatacagttctcaatcccacccaaagcaggtatgtcaataaatcacatattcctaggtgatacccaaatgctacagagtggaacactcagacctgagatttgcaaaaagcagatgtaaatatatgcattcaaacatcagggcttactatgaggtaggtggtatatacatgtcacaaataaaaatacagttacaactcagggtcacaaaaaatgcatcttccaatgcatatttttattatggtaaaatatacataaatataattcaccattttaacatttaattcatattaaatacgtacaaatcagtgacatttagtacattcacagtgttgtgccaccatcaccactatttagttccagaacatttgcatcatcaatacattgtctagagacaagactatcctgggtaggcagaaaccatagatcttttgtgtttacagctatggaaaccaactgtaccataaagatagttcactgagttttaaagccaagccacatcttatttttccaaggtttaatttagtgagagggcagcattagtgtggagtggcatgcttttgccctatcgtggaatttacacatcagaatgtgcaggatccaagtctgaaagtgttgccacccgtcacacaacatgggctttgtttgcttattccatgaagcagcagctatagaccttaccatggaaacatgaagagaccctgcacccctttccttaaggattgctgcaagagttacctgttgagcaggattgactggtgatgtttcattctgaccttgtcccaagctctccatctctagatctggggactgactgttgagctgatggggaaagaaaagctctcacacaaaccggaagccaaatgtcccctatctcttgaatgatcaagtcacttttgacaacatccaggtgaatataaaaacttaataaagctgtggaaaggaactcttaatcttcttttctgctacttaggttaaattcactagatcttgattaggaatcaaaattcgaattgggacatgttcaaattctttcttgtggtagttgcctatactgtcatcgctgctgttggttgagcatttgtggtgtaccacgctgtgtgctcaagggtattacattcatcttctcatttaatcctcacaacaatctgaagaaggtaggtattacaattcccacttcatagaaacagaaactgaggttcagagaggttaagtcatttgcccaaatggctgagccaaagcctaccatgtacctaacctttattttctttcccgaacataccaggctgtctcctcataacttccaagcatgcacttaaaactccacatgaatacaaggttcatgggacttggtattcatagaaagggaggcagaaagctggtctgttcctgataggcttgtaatttaatatcattctgttcatgtgctttggatggaagcacatctggcatatgatgctaatcagtggttcccatacccctggcttcctaattttaatgtttgctcacagcatagtagattgacatcaaatagtggccgatgatgatgaaaataaaggtcaaataagttgagccaataacagccgcttttttccttctgtctgcgtatacaaagcactgtcatgcacacaatctattctgaccctcacaacaacccataagggtgtaaatagtatttccattttacaaatgaggatcacacaaactactacatggcagagcagatactccaactcatgtcttctggttgaagcctattgctttttcttttctaaacactttccctcagcaagttggaattagacttcacaagtctccttcagagaacacaaatcttttcttattccattcctgtttggttgcctacgtccaatctccccctccccagagatgccaaaaaaaaaatcctttaaggtatttgggagccaaactcaacttgttaaaatctcaaattatggagacaatcagcagacacaacctaaccccaattattttggcaggaaggttggtttagaggcagatccagcaatctgctttgggccactctgggtggggtaggtgaaataagattggtcactgttaactaattttaatattggattggccattggttatcactgattaccattctcccctggattttcacccaggactcaaaacttggttctgctaaccctgttcctttatgaggaaccttttaaagattcctttataaggtgggagttttttttctatgaacctataggggagaaaaaagatcagcagaagtcattacttttttttttttttttttttttttttgagagagagtctcactccattgcccaggctggagtgcagtggtgctatctcggctcactgcaacctccgcctcctgggttcaagcaattctcctgcctcagcctcccgagtagctgggattgcaggtgcccaccaccacacccggctaatttttgtatttttagtaaagacagggtttcaccatgttggccaggctggtctccaactcccaatctcaggtgatcctattgcctcgggctcccaaagtgctgggattacaggagtgagccaccatgcctggccagaagtggttacttctgtagacaaaagaataatgctacttaatcaggctttctgtgtgacaagaaagagaaagaaaataaagaagtttcaattcatccaattcttaataagaaatatgtaaataaaattttttaaaattacacttcattttaatgttgtatcagtcaaggtccctgcaagagatggatggtatggtacactcaaactgggtaacacaggagagttttcagaaagcaactaaatccaaaatactatcaaggaatcaatataaaaattgttaatatttttctcatactaaattttcaaaatattttgtgtctattacatttacagcacatcttaattaggactagctgtgtgttcacctcacatgtggcttgtagctaccatactggacagcacatgtccaaaaaaatacacgtaaagttaaagtttaaaagacacaggaactaagccctcattgtctttcccttgggaggtagtttaaagagctatagatgctgtaacattcttgctattatttattatatatgacattattcctaaaaaagcttttgagatcctaggttgtattcctcaggttttgttgccttcccatgaagatgtgaaggcagggatgcctgttattcagtccaagatgcatgacaagagaccttgggaaagtttcatctggatttaaagattaattcttgatgcttacattccatactcaaaatgtaaatttgaatattaaaataaagatgattttttttttggagctagtcttgctctgttgcccaggctggaatgcagtggcatgatcatggctcactgcagcctcgacctcccaagctcaagcaaggctacaggtgtgcacctaagtagctaggactacaggtgtgcaccaccatgtctagctatttttttttctgtagagacagggttttcctatgttgtccaggctggtctcgaactcctgccctcaagcaatcctcctgccttggcctcccaaagtgttgagattacaggcgtaagccactgcacctggccaagatgaatattttaatagctcacagaacaaagtttgccacataatgataaaattactatgaaaatatattccctttattgtcagtttaaaagatgaactgagtttcacccaaactggtctggcccctctctgattcaaataccaatagttgctctgattcaaattccaactgttagaacatgacagctgctcataactagctttgcttactaaccatgtttctttccatttgtattaggtcctttactttttataacagcctcaaagtttcatgaattgctgcagtaaacattgattttcatgtttgtgagtctgcaagccagctgggcagctctacttcaggtggtaagggtggatcagacctattccatatacctcttgttctccttgtccagtggtttctagggatatgttctcatgatgaaccccgcagaggctcgtgaaagtgagaggaaactaggatgcctcttaaggtcttggtcaggatggggtctcctgtcacttctgtcacaggctattgtaagtcatatgagcaagctcaataaaatataaacaagtcagataaacagtgggaggaatggcaaagtcatatggccaaggccatgagtgattaattttaacacaggaaaaaagtaaagcattaaatgcgattatttaatatacaatgtcttattaactgaaatataaaatgtgtttactgtaaaatataatctgtttatctcaccaaagaaatattatctttaaaaaatgtcattacttctaagacatcatcagtctgcaacttctttccatagccttaatcaggatgctgtggcagctcccacattagcctcgcattctaaactggtagatgtcctaggaaaccatacatctatgtatttttcttattttatacgtttaggacaatgtatagctaattacccaactttttatttgcatacaaatctaatacaactgaacacaatcagttttatcacaggtataatggatttttcaatagtgaggaggtgcctccatgagccttctctttagaaaagtggcattcaagactcttcatttgaagtgaagattgctatgtcttttgcattgctctattttacataaattaagttataaattgacactataatcaactgacaccatgatcagtgatgatgatcaccctcatcagcactagagttgacttgtttttataacccctttgcatgtatgttgaatagcaaagttcatcagagaacatgtattagtcaatggtaagtaagatactctcatctaagaaataacatcacctcttctaatgaagttctaagaagagagggaagaaaaagtcttgggagctagtcagggaatagtgtgtatttgcaattacctaaactgaactctaccattactcctaacccagttcctcctcctgtgttttacatgattaatgccacccctgcctcaatgaaccaagatcagctccatcactgggacctccccattctgcctgtgcaatatttttcttttttatttctccttctaatattactgttattgctccagtaaagagctgtaatatattttacctggactgataccaggaatggtggtgttgcttccaatctgttgctgctagattaatctttgcaaagcacaggcttaatttcattgctgctcaactaaaaccactggtggctttccattgcctacaaaataaagtcaacctccccatcagacattcaaggctttcaatgatccatggccgccagctctctccaggctcatatcccactccactcctctgatgtttcctacactacactacactatactacactacagccaggtagaatgactgttcacccaacaccactcaggttgtcttctcaacttggaatactcttgcaccttcaaagctcatttcaaatgccccttcatttgtgaagccttctccaaatttccaagtcagaatgtctcttccttgtgctaccacaaccctttaactgagcctccattagtgcactgagaccattctgttcagtgtctgggtgaagcttcctggtgaaaaatatgttacctatttctttctgaaaagttggattcagggatattatcacggacctaaggtaatagttctagccaacctccctgtccactgccaggccgactacaaacccttctgttgctggcgagctggtccgcaccactagttctgcttcactctatttatctcttgatgtaaccatcttctttctccaggttttaagaaccagcccaactcctggttccctgatgaagcttttattcccctagccacatggaacttttcctttttggaacatgcctttagtttctgtgtagtttgccatgcagcacttcattgtacacattattaaaacagaattttaaggattagaatgaaccttaaaagatcatgcatctcaaaatttaatgtacatacaaattacccagggattttgttgaaataaaaattatttaattttaattaatataaataattcagtaggtctggggtgaggcctgaggttttacatttccaacaagctgccaggtaaagccaatacatctgtccaggaatcacactttgcgtatcaaaggtctagatgacattatcattccaaagagtttcttttacaggctctcagatcagtgttcatccactacctgactactgtcattcacaggcattctgttccacagcaggccagctaacgtggtatttacaaagctcactcctcttatacaacaatccaagtgtttcttttgtcagttgtctgtgccccaggagatccctctctgccttgccttgccctctgcctttggagaccagcacctcatactcagtgaaggcctggagtgcttaagagggatttcttccagctctcttgccctggtcttcagtgtattagatgtattacctccatgctctcagtagaggcccataggaaagagtaggtaggttatgccagctcacacgcatcctttaaaaatggtttagaagtttagctggtttcttattactcctgtctatggatgtttccttctgtcactctactagggatgaaacagctaatcatgttcaatagttacatttagattggtttttaaaaactatgattgtattagttcgtttccatgctgctgataaagacatatctgagactggaaacaaaaagggtttaattggacttacagttccacatggctggggaggcctcaaaatcaggtgggaggcaaaaggtacttcttacgtggtggcatcaagagcaaaatgaggaagaagcaaaagcagaaactcttcataaacccaccagatcttgtgggacttattatcacgagaatagcacagaaaagactggcctccatgattcaattacctcccactgcgtccctcccacaacatgtgggaattctgggagatacaattcaagttgagatttgggtggggacacagccaaaccatatcattcctccctgggctcctccaaatttcataatcctcacatttcaaaaccaatcattccttcccaacagttccccaaagtcttaactcatttcagcattaacccaaaagtccacagtccaaagtctcatctgagacaaggcaagtcccttccacttacaagcctgtaaaagcaagctagttacctcctagatacaatggggggtacaggtattgggtaaatacagctgttccaaatgagagaaattggccaaaacaaaggggttacagggtccatgcaagtctgaaatccagtggggcagtcaaattttaaagctccataatgatctcctttgactccatgtctcacattcaggtcatgctgatgcaagagataggttcccatggtcttgtgcagctccgcccctgtggctttgcagagtacagcctccctcctggctgctttctcaggctgatgttgagtgtctgtagcttttccaggcacaagatgcaagttggtggttgatctaccattctggggtctaccattctggggtctaccgttctgggactgtggccttcttctcacagctccactaggcagtgccccaacagggactctgtgtgggggctctgccccacatttcccttccacactgccctaggagaggttccccatgagggctctgcccctgcagcaaacttttgcctggacatccaggtgtttccatatatattctgaaatctaggcagaggttcccaaatctcaattcttgacatctctgcacccacaggctcaacatcacatggaagctgccaatgcttggggcctctaccctctgaagccacagcccaagctctatgttggctcctttcagccatggctggagcagctgggacacagggcaccaagtccctaggctgcacacagcacagagaccctgggcccagcccacaaaaccactttttcctcctgggcctctgggcctgtgatgggaggggctgccatgaaggtctctgacatgacctggagacattttccccatggtcttggggattaacattaggctccttgctgcttatgcaaatttctgcagccagcttgaatttctccttaaaaaaaatgggtttttcttttctactgcatcatcaggctgcagattttccacatttatgctcttgtttcccttttaaaacagaatgtttttaacagcacccaagtcaccttttgaatgctttgctgcttagaaatttattccaccagataccctaagtcatctctctcaagctctaagttccacaaatctctagggcaagggtgaaatgctgccagtctccttgctaaaacataacaagggtcacctttacttcagttcccaacaaggtcttcatctccatctgagaccacctcagcctggaccttattgttcatatcactatcagtatttttgtcaatgccattcacagtctctaggaggttccaaactttcctacattttcctatcttcttctgagccctccagattatttcaacacccagttccaaagttgcttccacattttcgggtatcttttcagcaatgccccactctactggtactattagtccattttcatgctgctgataaagacatacctgagactgggaacaaaaagaggtttaattggacttatagttccacctggctggggaggcctcagaatcatggcaggaggtgaaaggcatttcttacacggcagcagcaagagaaaaatgaagaagcagcaaaagcagaaacccctgataaaaccatcagatctcgtgagacttattcactatcacaagaatagcatgggaaagaccagcccccttgattcaattacctccccctgggtcctgtgggaattctggaaggtacaattcaagttgagatttgggtggggacacagccaaaccatatcaatgattttgtactttaaccagctgaatggaagtacaatctcttgctatatgacacaataattatttgcaaaatgagtaaacatatcataaggaaattatttttacaaggtttgaaacctgaaatgcagtctattatcatacataactaaaaatagagcctcaataaacagattcccagttttgaaaatgcaacatttgtactccacattgtcagttttcttaggtatatttataaatactcctataaaaatgtaaagaaacacataatgtagattgctaattttataataacacaagttgattttgacatccaacttattaattatgaaatgacttttggcctagtaacaatgaaaatgggggcaaatacagataaatggtaattcttagaatgaactactcagcaccaattctaagtttttcttgatggtaaatcataatgttccctttctcctcggttctgcaatctataggcataccataattgtaatcaatagcttaaaaatatgtctctctgtcctattctgtatctgtatctcttggatttttacctttgcaatagtcaactgaaccatcttcttggagtactcatgaagatggaagtctacatggagaatacaggatgaatccactctgtctcctgcagtgaagtctgtttgaaggatgtatttggctgtcttctggacaggccattctaataacagaaacaaacaagttattttaaaacttattggaatattcaaatattaaccaaagtagaaaaatataatacacatccatgtgcccatcacagaacttcactgattatcatcatttagccagtcttgaagaagcaagtgctaattacaatcacaaatgaaacaagattcagacttcatgaagagcactgcgctataataaaagaagaaatgagcacatacattcttttactgacagtcaaatggtgaaggtgggcagaatcattatgtgatgcaacatggcaaaagtatacagacagtgcatccagaggaaggcaccttgctgaatgactagaatggaagtaggagacattttgcaggcccccttcatcctgcagggagaaccagaaccacagcagctctatttgcctattcctctttaaattacaaagttaaaatttgggagtagtagaaaatcaattggttatcttatagagtctcctagaatatttcattggcattgagaaggtggaaaatgcaaattatatactttaaaatgtaatttttgcttttcacatatgcttaaagcctaaaacctcttaataaacttcttctgaaatata

SEQ ID NO: 2 - protein, 510 aa, Homo sapiens
MEDTKESNVKTFCSKNILAILGFSSIIAVIALLAVGLTQNKALPENVKYGIVLDAGSSHTSLYIYKWPAEKENDTGVVHQVEECRVKGPGISKFVQKVNEIGIYLTDCMERAREVIPRSQHQETPVYLGATAGMRLLRMESEELADRVLDVVERSLSNYPFDFQGARIITGQEEGAYGWITINYLLGKFSQKTRWFSIVPYETNNQETFGALDLGGASTQVTFVPQNQTIESPDNALQFRLYGKDYNVYTHSFLCYGKDQALWQKLAKDIQVASNEILRDPCFHPGYKKVVNVSDLYKTPCTKRFEMTLPFQQFEIQGIGNYQQCHQSILELFNTSYCPYSQCAFNGIFLPPLQGDFGAFSAFYFVMKFLNLTSEKVSQEKVTEMMKKFCAQPWEEIKTSYAGVKEKYLSEYCFSGTYILSLLLQGYHFTADSWEHIHFIGKIQGSDAGWTLGYMLNLTNMIPAEQPLSTPLSHSTYVFLMVLFSLVLFTVAIIGLLIFHKPSYFWKDMV

SEQ ID NO: 3 - DNA, 12630 bp, Homo sapiens
attctgcagtctcctgtgtacgtgtaaaattatgatcaaataaatttgtatgccttttctcctattaacctgccttttttgtcagcgattgtcagtgaaacttcagagggcaaaggggaagttttccttggcccctccagttttggtgctgtgaacaggataccaaagctgctctgttcttctggaagctgcaatgaagggaaccaaggacctgacaagccagcagaaggagtctaacgtgaagacattttgctccaagaatatcctagccatccttggcttctcctctatcatagctgtgatagctttgcttgctgtggggttgacccagaacaaagcattgccagaaaacgttaagtatgggattgtgctggatgcgggttcttctcacacaagtttatacatctataagtggccagcagaaaaggagaatgacacaggcgtggtgcatcaagtagaagaatgcagggttaaaggtcctggaatctcaaaatttgttcagaaagtaaatgaaataggcatttacctgactgattgcatggaaagagctagggaagtgattccaaggtcccagcaccaagagacacccgtttacctgggagccacggcaggcatgcggttgctcaggatggaaagtgaagagttggcagacagggttctggatgtggtggagaggagcctcagcaactacccctttgacttccagggtgccaggatcattactggccaagaggaaggtgcctatggctggattactatcaactatctgctgggcaaattcagtcagaaaacaaggtggttcagcatagtcccatatgaaaccaataatcaggaaacctttggagctttggaccttgggggagcctctacacaagtcacttttgtaccccaaaaccagactatcgagtccccagataatgctctgcaatttcgcctctatggcaaggactacaatgtctacacacatagcttcttgtgctatgggaaggatcaggcactctggcagaaactggccaaggacattcaggttgcaagtaatgaaattctcagggacccatgctttcatcctggatataagaaggtagtgaacgtaagtgacctttacaagaccccctgcaccaagagatttgagatgactcttccattccagcagtttgaaatccagggtattggaaactatcaacaatgccatcaaagcatcctggagctcttcaacaccagttactgcccttactcccagtgtgccttcaatgggattttcttgccaccactccagggggattttggggcattttcagctttttactttgtgatgaagtttttaaacttgacatcagagaaagtctctcaggaaaaggtgactgagatgatgaaaaagttctgtgctcagccttgggaggagataaaaacatcttacgctggagtaaaggagaagtacctgagtgaatactgcttttctggtacctacattctctccctccttctgcaaggctatcatttcacagctgattcctgggagcacatccatttcattggcaagatccagggcagcgacgccggctggactttgggctacatgctgaacctgaccaacatgatcccagctgagcaaccattgtccacacctctctcccactccacctatgtcttcctcatggttctattctccctggtccttttcacagtggccatcataggcttgcttatctttcacaagccttcatatttctggaaagatatggtatagcaaaagcagctgaaatatgctggctggagtgaggaaaaaaatcgtccagggagcattttcctccatcgcagtgttcaaggccatccttccctgtctgccagggccagtcttgacgagtgtgaagcttccttggcttttactgaagcctttcttttggaggtattcaatatcctttgcctcaaggacttcggcagatactgtctctttcatgagtttttcccagctacacctttctcctttgtactttgtgcttgtataggttttaaagacctgacacctttcataatctttgctttataaaagaacaatattgactttgtctagaagaactgagagtcttgagtcctgtgataggaggctgagctggctgaaagaagaatctcaggaactggttcagttgtactctttaagaacccctttctctctcctgtttgccatccattaagaaagccatatgatgcctttggagaaggcagacacacattccattcccagcctgctctgtgggtaggagaattttctacagtaggcaaatatgtgctaaagccaaagagttttataaggaaatatatgtgctcatgcagtcaatacagttctcaatcccacccaaagcaggtatgtcaataaatcacatattcctaggtgatacccaaatgctacagagtggaacactcagacctgagatttgcaaaaagcagatgtaaatatatgcattcaaacatcagggcttactatgaggtaggtggtatatacatgtcacaaataaaaatacagttacaactcagggtcacaaaaaatgcatcttccaatgcatatttttattatggtaaaatatacataaatataattcaccattttaacatttaattcatattaaatacgtacaaatcagtgacatttagtacattcacagtgttgtgccaccatcaccactatttagttccagaacatttgcatcatcaatacattgtctagagacaagactatcctgggtaggcagaaaccatagatcttttgtgtttacagctatggaaaccaactgtaccataaagatagttcactgagttttaaagccaagccacatcttatttttccaaggtttaatttagtgagagggcagcattagtgtggagtggcatgcttttgccctatcgtggaatttacacatcagaatgtgcaggatccaagtctgaaagtgttgccacccgtcacacaacatgggctttgtttgcttattccatgaagcagcagctatagaccttaccatggaaacatgaagagaccctgcacccctttccttaaggattgctgcaagagttacctgttgagcaggattgactggtgatgtttcattctgaccttgtcccaagctctccatctctagatctggggactgactgttgagctgatggggaaagaaaagctctcacacaaaccggaagccaaatgtcccctatctcttgaatgatcaagtcacttttgacaacatccaggtgaatataaaaacttaataaagctgtggaaaggaactcttaatcttcttttctgctacttaggttaaattcactagatcttgattaggaatcaaaattcgaattgggacatgttcaaattctttcttgtggtagttgcctatactgtcatcgctgctgttggttgagcatttgtggtgtaccacgctgtgtgctcaagggtattacattcatcttctcatttaatcctcacaacaatctgaagaaggtaggtattacaattcccacttcatagaaacagaaactgaggttcagagaggttaagtcatttgcccaaatggctgagccaaagcctaccatgtacctaacctttattttctttcccgaacataccaggctgtctcctcataacttccaagcatgcacttaaaactccacatgaatacaaggttcatgggacttggtattcatagaaagggaggcagaaagctggtctgttcctgataggcttgtaatttaatatcattctgttcatgtgctttggatggaagcacatctggcatatgatgctaatcagtggttcccatacccctggcttcctaattttaatgtttgctcacagcatagtagattgacatcaaatagtggccgatgatgatgaaaataaaggtcaaataagttgagccaataacagccgcttttttccttctgtctgcgtatacaaagcactgtcatgcacacaatctattctgaccctcacaacaacccataagggtgtaaatagtatttccattttacaaatgaggatcacacaaactactacatggcagagcagatactccaactcatgtcttctggttgaagcctattgctttttcttttctaaacactttccctcagcaagttggaattagacttcacaagtctccttcagagaacacaaatcttttcttattccattcctgtttggttgcctacgtccaatctccccctccccagagatgccaaaaaaaaaatcctttaaggtatttgggagccaaactcaacttgttaaaatctcaaattatggagacaatcagcagacacaacctaaccccaattattttggcaggaaggttggtttagaggcagatccagcaatctgctttgggccactctgggtggggtaggtgaaataagattggtcactgttaactaattttaatattggattggccattggttatcactgattaccattctcccctggattttcacccaggactcaaaacttggttctgctaaccctgttcctttatgaggaaccttttaaagattcctttataaggtgggagttttttttctatgaacctataggggagaaaaaagatcagcagaagtcattacttttttttttttttttttttttttttgagagagagtctcactccattgcccaggctggagtgcagtggtgctatctcggctcactgcaacctccgcctcctgggttcaagcaattctcctgcctcagcctcccgagtagctgggattgcaggtgcccaccaccacacccggctaatttttgtatttttagtaaagacagggtttcaccatgttggccaggctggtctccaactcccaatctcaggtgatcctattgcctcgggctcccaaagtgctgggattacaggagtgagccaccatgcctggccagaagtggttacttctgtagacaaaagaataatgctacttaatcaggctttctgtgtgacaagaaagagaaagaaaataaagaagtttcaattcatccaattcttaataagaaatatgtaaataaaattttttaaaattacacttcattttaatgttgtatcagtcaaggtccctgcaagagatggatggtatggtacactcaaactgggtaacacaggagagttttcagaaagcaactaaatccaaaatactatcaaggaatcaatataaaaattgttaatatttttctcatactaaattttcaaaatattttgtgtctattacatttacagcacatcttaattaggactagctgtgtgttcacctcacatgtggcttgtagctaccatactggacagcacatgtccaaaaaaatacacgtaaagttaaagtttaaaagacacaggaactaagccctcattgtctttcccttgggaggtagtttaaagagctatagatgctgtaacattcttgctattatttattatatatgacattattcctaaaaaagcttttgagatcctaggttgtattcctcaggttttgttgccttcccatgaagatgtgaaggcagggatgcctgttattcagtccaagatgcatgacaagagaccttgggaaagtttcatctggatttaaagattaattcttgatgcttacattccatactcaaaatgtaaatttgaatattaaaataaagatgattttttttttggagctagtcttgctctgttgcccaggctggaatgcagtggcatgatcatggctcactgcagcctcgacctcccaagctcaagcaaggctacaggtgtgcacctaagtagctaggactacaggtgtgcaccaccatgtctagctatttttttttctgtagagacagggttttcctatgttgtccaggctggtctcgaactcctgccctcaagcaatcctcctgccttggcctcccaaagtgttgagattacaggcgtaagccactgcacctggccaagatgaatattttaatagctcacagaacaaagtttgccacataatgataaaattactatgaaaatatattccctttattgtcagtttaaaagatgaactgagtttcacccaaactggtctggcccctctctgattcaaataccaatagttgctctgattcaaattccaactgttagaacatgacagctgctcataactagctttgcttactaaccatgtttctttccatttgtattaggtcctttactttttataacagcctcaaagtttcatgaattgctgcagtaaacattgattttcatgtttgtgagtctgcaagccagctgggcagctctacttcaggtggtaagggtggatcagacctattccatatacctcttgttctccttgtccagtggtttctagggatatgttctcatgatgaaccccgcagaggctcgtgaaagtgagaggaaactaggatgcctcttaaggtcttggtcaggatggggtctcctgtcacttctgtcacaggctattgtaagtcatatgagcaagctcaataaaatataaacaagtcagataaacagtgggaggaatggcaaagtcatatggccaaggccatgagtgattaattttaacacaggaaaaaagtaaagcattaaatgcgattatttaatatacaatgtcttattaactgaaatataaaatgtgtttactgtaaaatataatctgtttatctcaccaaagaaatattatctttaaaaaatgtcattacttctaagacatcatcagtctgcaacttctttccatagccttaatcaggatgctgtggcagctcccacattagcctcgcattctaaactggtagatgtcctaggaaaccatacatctatgtatttttcttattttatacgtttaggacaatgtatagctaattacccaactttttatttgcatacaaatctaatacaactgaacacaatcagttttatcacaggtataatggatttttcaatagtgaggaggtgcctccatgagccttctctttagaaaagtggcattcaagactcttcatttgaagtgaagattgctatgtcttttgcattgctctattttacataaattaagttataaattgacactataatcaactgacaccatgatcagtgatgatgatcaccctcatcagcactagagttgacttgtttttataacccctttgcatgtatgttgaatagcaaagttcatcagagaacatgtattagtcaatggtaagtaagatactctcatctaagaaataacatcacctcttctaatgaagttctaagaagagagggaagaaaaagtcttgggagctagtcagggaatagtgtgtatttgcaattacctaaactgaactctaccattactcctaacccagttcctcctcctgtgttttacatgattaatgccacccctgcctcaatgaaccaagatcagctccatcactgggacctccccattctgcctgtgcaatatttttcttttttatttctccttctaatattactgttattgctccagtaaagagctgtaatatattttacctggactgataccaggaatggtggtgttgcttccaatctgttgctgctagattaatctttgcaaagcacaggcttaatttcattgctgctcaactaaaaccactggtggctttccattgcctacaaaataaagtcaacctccccatcagacattcaaggctttcaatgatccatggccgccagctctctccaggctcatatcccactccactcctctgatgtttcctacactacactacactatactacactacagccaggtagaatgactgttcacccaacaccactcaggttgtcttctcaacttggaatactcttgcaccttcaaagctcatttcaaatgccccttcatttgtgaagccttctccaaatttccaagtcagaatgtctcttccttgtgctaccacaaccctttaactgagcctccattagtgcactgagaccattctgttcagtgtctgggtgaagcttcctggtgaaaaatatgttacctatttctttctgaaaagttggattcagggatattatcacggacctaaggtaatagttctagccaacctccctgtccactgccaggccgactacaaacccttctgttgctggcgagctggtccgcaccactagttctgcttcactctatttatctcttgatgtaaccatcttctttctccaggttttaagaaccagcccaactcctggttccctgatgaagcttttattcccctagccacatggaacttttcctttttggaacatgcctttagtttctgtgtagtttgccatgcagcacttcattgtacacattattaaaacagaattttaaggattagaatgaaccttaaaagatcatgcatctcaaaatttaatgtacatacaaattacccagggattttgttgaaataaaaattatttaattttaattaatataaataattcagtaggtctggggtgaggcctgaggttttacatttccaacaagctgccaggtaaagccaatacatctgtccaggaatcacactttgcgtatcaaaggtctagatgacattatcattccaaagagtttcttttacaggctctcagatcagtgttcatccactacctgactactgtcattcacaggcattctgttccacagcaggccagctaacgtggtatttacaaagctcactcctcttatacaacaatccaagtgtttcttttgtcagttgtctgtgccccaggagatccctctctgccttgccttgccctctgcctttggagaccagcacctcatactcagtgaaggcctggagtgcttaagagggatttcttccagctctcttgccctggtcttcagtgtattagatgtattacctccatgctctcagtagaggcccataggaaagagtaggtaggttatgccagctcacacgcatcctttaaaaatggtttagaagtttagctggtttcttattactcctgtctatggatgtttccttctgtcactctactagggatgaaacagctaatcatgttcaatagttacatttagattggtttttaaaaactatgattgtattagttcgtttccatgctgctgataaagacatatctgagactggaaacaaaaagggtttaattggacttacagttccacatggctggggaggcctcaaaatcaggtgggaggcaaaaggtacttcttacgtggtggcatcaagagcaaaatgaggaagaagcaaaagcagaaactcttcataaacccaccagatcttgtgggacttattatcacgagaatagcacagaaaagactggcctccatgattcaattacctcccactgcgtccctcccacaacatgtgggaattctgggagatacaattcaagttgagatttgggtggggacacagccaaaccatatcattcctccctgggctcctccaaatttcataatcctcacatttcaaaaccaatcattccttcccaacagttccccaaagtcttaactcatttcagcattaacccaaaagtccacagtccaaagtctcatctgagacaaggcaagtcccttccacttacaagcctgtaaaagcaagctagttacctcctagatacaatggggggtacaggtattgggtaaatacagctgttccaaatgagagaaattggccaaaacaaaggggttacagggtccatgcaagtctgaaatccagtggggcagtcaaattttaaagctccataatgatctcctttgactccatgtctcacattcaggtcatgctgatgcaagagataggttcccatggtcttgtgcagctccgcccctgtggctttgcagagtacagcctccctcctggctgctttctcaggctgatgttgagtgtctgtagcttttccaggcacaagatgcaagttggtggttgatctaccattctggggtctaccattctggggtctaccgttctgggactgtggccttcttctcacagctccactaggcagtgccccaacagggactctgtgtgggggctctgccccacatttcccttccacactgccctaggagaggttccccatgagggctctgcccctgcagcaaacttttgcctggacatccaggtgtttccatatatattctgaaatctaggcagaggttcccaaatctcaattcttgacatctctgcacccacaggctcaacatcacatggaagctgccaatgcttggggcctctaccctctgaagccacagcccaagctctatgttggctcctttcagccatggctggagcagctgggacacagggcaccaagtccctaggctgcacacagcacagagaccctgggcccagcccacaaaaccactttttcctcctgggcctctgggcctgtgatgggaggggctgccatgaaggtctctgacatgacctggagacattttccccatggtcttggggattaacattaggctccttgctgcttatgcaaatttctgcagccagcttgaatttctccttaaaaaaaatgggtttttcttttctactgcatcatcaggctgcagattttccacatttatgctcttgtttcccttttaaaacagaatgtttttaacagcacccaagtcaccttttgaatgctttgctgcttagaaatttattccaccagataccctaagtcatctctctcaagctctaagttccacaaatctctagggcaagggtgaaatgctgccagtctccttgctaaaacataacaagggtcacctttacttcagttcccaacaaggtcttcatctccatctgagaccacctcagcctggaccttattgttcatatcactatcagtatttttgtcaatgccattcacagtctctaggaggttccaaactttcctacattttcctatcttcttctgagccctccagattatttcaacacccagttccaaagttgcttccacattttcgggtatcttttcagcaatgccccactctactggtactattagtccattttcatgctgctgataaagacatacctgagactgggaacaaaaagaggtttaattggacttatagttccacctggctggggaggcctcagaatcatggcaggaggtgaaaggcatttcttacacggcagcagcaagagaaaaatgaagaagcagcaaaagcagaaacccctgataaaaccatcagatctcgtgagacttattcactatcacaagaatagcatgggaaagaccagcccccttgattcaattacctccccctgggtcctgtgggaattctggaaggtacaattcaagttgagatttgggtggggacacagccaaaccatatcaatgattttgtactttaaccagctgaatggaagtacaatctcttgctatatgacacaataattatttgcaaaatgagtaaacatatcataaggaaattatttttacaaggtttgaaacctgaaatgcagtctattatcatacataactaaaaatagagcctcaataaacagattcccagttttgaaaatgcaacatttgtactccacattgtcagttttcttaggtatatttataaatactcctataaaaatgtaaagaaacacataatgtagattgctaattttataataacacaagttgattttgacatccaacttattaattatgaaatgacttttggcctagtaacaatgaaaatgggggcaaatacagataaatggtaattcttagaatgaactactcagcaccaattctaagtttttcttgatggtaaatcataatgttccctttctcctcggttctgcaatctataggcataccataattgtaatcaatagcttaaaaatatgtctctctgtcctattctgtatctgtatctcttggatttttacctttgcaatagtcaactgaaccatcttcttggagtactcatgaagatggaagtctacatggagaatacaggatgaatccactctgtctcctgcagtgaagtctgtttgaaggatgtatttggctgtcttctggacaggccattctaataacagaaacaaacaagttattttaaaacttattggaatattcaaatattaaccaaagtagaaaaatataatacacatccatgtgcccatcacagaacttcactgattatcatcatttagccagtcttgaagaagcaagtgctaattacaatcacaaatgaaacaagattcagacttcatgaagagcactgcgctataataaaagaagaaatgagcacatacattcttttactgacagtcaaatggtgaaggtgggcagaatcattatgtgatgcaacatggcaaaagtatacagacagtgcatccagaggaaggcaccttgctgaatgactagaatggaagtaggagacattttgcaggcccccttcatcctgcagggagaaccagaaccacagcagctctatttgcctattcctctttaaattacaaagttaaaatttgggagtagtagaaaatcaattggttatcttatagagtctcctagaatatttcattggcattgagaaggtggaaaatgcaaattatatactttaaaatgtaatttttgcttttcacatatgcttaaagcctaaaacctcttaataaacttcttctgaaatata

SEQ ID NO: 4 - protein, 517 aa, Homo sapiens
MKGTKDLTSQQKESNVKTFCSKNILAILGFSSIIAVIALLAVGLTQNKALPENVKYGIVLDAGSSHTSLYIYKWPAEKENDTGVVHQVEECRVKGPGISKFVQKVNEIGIYLTDCMERAREVIPRSQHQETPVYLGATAGMRLLRMESEELADRVLDVVERSLSNYPFDFQGARIITGQEEGAYGWITINYLLGKFSQKTRWFSIVPYETNNQETFGALDLGGASTQVTFVPQNQTIESPDNALQFRLYGKDYNVYTHSFLCYGKDQALWQKLAKDIQVASNEILRDPCFHPGYKKVVNVSDLYKTPCTKRFEMTLPFQQFEIQGIGNYQQCHQSILELFNTSYCPYSQCAFNGIFLPPLQGDFGAFSAFYFVMKFLNLTSEKVSQEKVTEMMKKFCAQPWEEIKTSYAGVKEKYLSEYCFSGTYILSLLLQGYHFTADSWEHIHFIGKIQGSDAGWTLGYMLNLTNMIPAEQPLSTPLSHSTYVFLMVLFSLVLFTVAIIGLLIFHKPSYFWKDMV

SEQ ID NO: 5 - DNA, 12515 bp, Homo sapiens
cctgttgctctttgctctaatgagccttgagaaaggattgctggtcatgggaccagaggctttatggggagggaagaactgttcttgactttcagtttttcgagcgggtttcaagagtctaacgtgaagacattttgctccaagaatatcctagccatccttggcttctcctctatcatagctgtgatagctttgcttgctgtggggttgacccagaacaaagcattgccagaaaacgttaagtatgggattgtgctggatgcgggttcttctcacacaagtttatacatctataagtggccagcagaaaaggagaatgacacaggcgtggtgcatcaagtagaagaatgcagggttaaaggtcctggaatctcaaaatttgttcagaaagtaaatgaaataggcatttacctgactgattgcatggaaagagctagggaagtgattccaaggtcccagcaccaagagacacccgtttacctgggagccacggcaggcatgcggttgctcaggatggaaagtgaagagttggcagacagggttctggatgtggtggagaggagcctcagcaactacccctttgacttccagggtgccaggatcattactggccaagaggaaggtgcctatggctggattactatcaactatctgctgggcaaattcagtcagaaaacaaggtggttcagcatagtcccatatgaaaccaataatcaggaaacctttggagctttggaccttgggggagcctctacacaagtcacttttgtaccccaaaaccagactatcgagtccccagataatgctctgcaatttcgcctctatggcaaggactacaatgtctacacacatagcttcttgtgctatgggaaggatcaggcactctggcagaaactggccaaggacattcaggttgcaagtaatgaaattctcagggacccatgctttcatcctggatataagaaggtagtgaacgtaagtgacctttacaagaccccctgcaccaagagatttgagatgactcttccattccagcagtttgaaatccagggtattggaaactatcaacaatgccatcaaagcatcctggagctcttcaacaccagttactgcccttactcccagtgtgccttcaatgggattttcttgccaccactccagggggattttggggcattttcagctttttactttgtgatgaagtttttaaacttgacatcagagaaagtctctcaggaaaaggtgactgagatgatgaaaaagttctgtgctcagccttgggaggagataaaaacatcttacgctggagtaaaggagaagtacctgagtgaatactgcttttctggtacctacattctctccctccttctgcaaggctatcatttcacagctgattcctgggagcacatccatttcattggcaagatccagggcagcgacgccggctggactttgggctacatgctgaacctgaccaacatgatcccagctgagcaaccattgtccacacctctctcccactccacctatgtcttcctcatggttctattctccctggtccttttcacagtggccatcataggcttgcttatctttcacaagccttcatatttctggaaagatatggtatagcaaaagcagctgaaatatgctggctggagtgaggaaaaaaatcgtccagggagcattttcctccatcgcagtgttcaaggccatccttccctgtctgccagggccagtcttgacgagtgtgaagcttccttggcttttactgaagcctttcttttggaggtattcaatatcctttgcctcaaggacttcggcagatactgtctctttcatgagtttttcccagctacacctttctcctttgtactttgtgcttgtataggttttaaagacctgacacctttcataatctttgctttataaaagaacaatattgactttgtctagaagaactgagagtcttgagtcctgtgataggaggctgagctggctgaaagaagaatctcaggaactggttcagttgtactctttaagaacccctttctctctcctgtttgccatccattaagaaagccatatgatgcctttggagaaggcagacacacattccattcccagcctgctctgtgggtaggagaattttctacagtaggcaaatatgtgctaaagccaaagagttttataaggaaatatatgtgctcatgcagtcaatacagttctcaatcccacccaaagcaggtatgtcaataaatcacatattcctaggtgatacccaaatgctacagagtggaacactcagacctgagatttgcaaaaagcagatgtaaatatatgcattcaaacatcagggcttactatgaggtaggtggtatatacatgtcacaaataaaaatacagttacaactcagggtcacaaaaaatgcatcttccaatgcatatttttattatggtaaaatatacataaatataattcaccattttaacatttaattcatattaaatacgtacaaatcagtgacatttagtacattcacagtgttgtgccaccatcaccactatttagttccagaacatttgcatcatcaatacattgtctagagacaagactatcctgggtaggcagaaaccatagatcttttgtgtttacagctatggaaaccaactgtaccataaagatagttcactgagttttaaagccaagccacatcttatttttccaaggtttaatttagtgagagggcagcattagtgtggagtggcatgcttttgccctatcgtggaatttacacatcagaatgtgcaggatccaagtctgaaagtgttgccacccgtcacacaacatgggctttgtttgcttattccatgaagcagcagctatagaccttaccatggaaacatgaagagaccctgcacccctttccttaaggattgctgcaagagttacctgttgagcaggattgactggtgatgtttcattctgaccttgtcccaagctctccatctctagatctggggactgactgttgagctgatggggaaagaaaagctctcacacaaaccggaagccaaatgtcccctatctcttgaatgatcaagtcacttttgacaacatccaggtgaatataaaaacttaataaagctgtggaaaggaactcttaatcttcttttctgctacttaggttaaattcactagatcttgattaggaatcaaaattcgaattgggacatgttcaaattctttcttgtggtagttgcctatactgtcatcgctgctgttggttgagcatttgtggtgtaccacgctgtgtgctcaagggtattacattcatcttctcatttaatcctcacaacaatctgaagaaggtaggtattacaattcccacttcatagaaacagaaactgaggttcagagaggttaagtcatttgcccaaatggctgagccaaagcctaccatgtacctaacctttattttctttcccgaacataccaggctgtctcctcataacttccaagcatgcacttaaaactccacatgaatacaaggttcatgggacttggtattcatagaaagggaggcagaaagctggtctgttcctgataggcttgtaatttaatatcattctgttcatgtgctttggatggaagcacatctggcatatgatgctaatcagtggttcccatacccctggcttcctaattttaatgtttgctcacagcatagtagattgacatcaaatagtggccgatgatgatgaaaataaaggtcaaataagttgagccaataacagccgcttttttccttctgtctgcgtatacaaagcactgtcatgcacacaatctattctgaccctcacaacaacccataagggtgtaaatagtatttccattttacaaatgaggatcacacaaactactacatggcagagcagatactccaactcatgtcttctggttgaagcctattgctttttcttttctaaacactttccctcagcaagttggaattagacttcacaagtctccttcagagaacacaaatcttttcttattccattcctgtttggttgcctacgtccaatctccccctccccagagatgccaaaaaaaaaatcctttaaggtatttgggagccaaactcaacttgttaaaatctcaaattatggagacaatcagcagacacaacctaaccccaattattttggcaggaaggttggtttagaggcagatccagcaatctgctttgggccactctgggtggggtaggtgaaataagattggtcactgttaactaattttaatattggattggccattggttatcactgattaccattctcccctggattttcacccaggactcaaaacttggttctgctaaccctgttcctttatgaggaaccttttaaagattcctttataaggtgggagttttttttctatgaacctataggggagaaaaaagatcagcagaagtcattacttttttttttttttttttttttttttgagagagagtctcactccattgcccaggctggagtgcagtggtgctatctcggctcactgcaacctccgcctcctgggttcaagcaattctcctgcctcagcctcccgagtagctgggattgcaggtgcccaccaccacacccggctaatttttgtatttttagtaaagacagggtttcaccatgttggccaggctggtctccaactcccaatctcaggtgatcctattgcctcgggctcccaaagtgctgggattacaggagtgagccaccatgcctggccagaagtggttacttctgtagacaaaagaataatgctacttaatcaggctttctgtgtgacaagaaagagaaagaaaataaagaagtttcaattcatccaattcttaataagaaatatgtaaataaaattttttaaaattacacttcattttaatgttgtatcagtcaaggtccctgcaagagatggatggtatggtacactcaaactgggtaacacaggagagttttcagaaagcaactaaatccaaaatactatcaaggaatcaatataaaaattgttaatatttttctcatactaaattttcaaaatattttgtgtctattacatttacagcacatcttaattaggactagctgtgtgttcacctcacatgtggcttgtagctaccatactggacagcacatgtccaaaaaaatacacgtaaagttaaagtttaaaagacacaggaactaagccctcattgtctttcccttgggaggtagtttaaagagctatagatgctgtaacattcttgctattatttattatatatgacattattcctaaaaaagcttttgagatcctaggttgtattcctcaggttttgttgccttcccatgaagatgtgaaggcagggatgcctgttattcagtccaagatgcatgacaagagaccttgggaaagtttcatctggatttaaagattaattcttgatgcttacattccatactcaaaatgtaaatttgaatattaaaataaagatgattttttttttggagctagtcttgctctgttgcccaggctggaatgcagtggcatgatcatggctcactgcagcctcgacctcccaagctcaagcaaggctacaggtgtgcacctaagtagctaggactacaggtgtgcaccaccatgtctagctatttttttttctgtagagacagggttttcctatgttgtccaggctggtctcgaactcctgccctcaagcaatcctcctgccttggcctcccaaagtgttgagattacaggcgtaagccactgcacctggccaagatgaatattttaatagctcacagaacaaagtttgccacataatgataaaattactatgaaaatatattccctttattgtcagtttaaaagatgaactgagtttcacccaaactggtctggcccctctctgattcaaataccaatagttgctctgattcaaattccaactgttagaacatgacagctgctcataactagctttgcttactaaccatgtttctttccatttgtattaggtcctttactttttataacagcctcaaagtttcatgaattgctgcagtaaacattgattttcatgtttgtgagtctgcaagccagctgggcagctctacttcaggtggtaagggtggatcagacctattccatatacctcttgttctccttgtccagtggtttctagggatatgttctcatgatgaaccccgcagaggctcgtgaaagtgagaggaaactaggatgcctcttaaggtcttggtcaggatggggtctcctgtcacttctgtcacaggctattgtaagtcatatgagcaagctcaataaaatataaacaagtcagataaacagtgggaggaatggcaaagtcatatggccaaggccatgagtgattaattttaacacaggaaaaaagtaaagcattaaatgcgattatttaatatacaatgtcttattaactgaaatataaaatgtgtttactgtaaaatataatctgtttatctcaccaaagaaatattatctttaaaaaatgtcattacttctaagacatcatcagtctgcaacttctttccatagccttaatcaggatgctgtggcagctcccacattagcctcgcattctaaactggtagatgtcctaggaaaccatacatctatgtatttttcttattttatacgtttaggacaatgtatagctaattacccaactttttatttgcatacaaatctaatacaactgaacacaatcagttttatcacaggtataatggatttttcaatagtgaggaggtgcctccatgagccttctctttagaaaagtggcattcaagactcttcatttgaagtgaagattgctatgtcttttgcattgctctattttacataaattaagttataaattgacactataatcaactgacaccatgatcagtgatgatgatcaccctcatcagcactagagttgacttgtttttataacccctttgcatgtatgttgaatagcaaagttcatcagagaacatgtattagtcaatggtaagtaagatactctcatctaagaaataacatcacctcttctaatgaagttctaagaagagagggaagaaaaagtcttgggagctagtcagggaatagtgtgtatttgcaattacctaaactgaactctaccattactcctaacccagttcctcctcctgtgttttacatgattaatgccacccctgcctcaatgaaccaagatcagctccatcactgggacctccccattctgcctgtgcaatatttttcttttttatttctccttctaatattactgttattgctccagtaaagagctgtaatatattttacctggactgataccaggaatggtggtgttgcttccaatctgttgctgctagattaatctttgcaaagcacaggcttaatttcattgctgctcaactaaaaccactggtggctttccattgcctacaaaataaagtcaacctccccatcagacattcaaggctttcaatgatccatggccgccagctctctccaggctcatatcccactccactcctctgatgtttcctacactacactacactatactacactacagccaggtagaatgactgttcacccaacaccactcaggttgtcttctcaacttggaatactcttgcaccttcaaagctcatttcaaatgccccttcatttgtgaagccttctccaaatttccaagtcagaatgtctcttccttgtgctaccacaaccctttaactgagcctccattagtgcactgagaccattctgttcagtgtctgggtgaagcttcctggtgaaaaatatgttacctatttctttctgaaaagttggattcagggatattatcacggacctaaggtaatagttctagccaacctccctgtccactgccaggccgactacaaacccttctgttgctggcgagctggtccgcaccactagttctgcttcactctatttatctcttgatgtaaccatcttctttctccaggttttaagaaccagcccaactcctggttccctgatgaagcttttattcccctagccacatggaacttttcctttttggaacatgcctttagtttctgtgtagtttgccatgcagcacttcattgtacacattattaaaacagaattttaaggattagaatgaaccttaaaagatcatgcatctcaaaatttaatgtacatacaaattacccagggattttgttgaaataaaaattatttaattttaattaatataaataattcagtaggtctggggtgaggcctgaggttttacatttccaacaagctgccaggtaaagccaatacatctgtccaggaatcacactttgcgtatcaaaggtctagatgacattatcattccaaagagtttcttttacaggctctcagatcagtgttcatccactacctgactactgtcattcacaggcattctgttccacagcaggccagctaacgtggtatttacaaagctcactcctcttatacaacaatccaagtgtttcttttgtcagttgtctgtgccccaggagatccctctctgccttgccttgccctctgcctttggagaccagcacctcatactcagtgaaggcctggagtgcttaagagggatttcttccagctctcttgccctggtcttcagtgtattagatgtattacctccatgctctcagtagaggcccataggaaagagtaggtaggttatgccagctcacacgcatcctttaaaaatggtttagaagtttagctggtttcttattactcctgtctatggatgtttccttctgtcactctactagggatgaaacagctaatcatgttcaatagttacatttagattggtttttaaaaactatgattgtattagttcgtttccatgctgctgataaagacatatctgagactggaaacaaaaagggtttaattggacttacagttccacatggctggggaggcctcaaaatcaggtgggaggcaaaaggtacttcttacgtggtggcatcaagagcaaaatgaggaagaagcaaaagcagaaactcttcataaacccaccagatcttgtgggacttattatcacgagaatagcacagaaaagactggcctccatgattcaattacctcccactgcgtccctcccacaacatgtgggaattctgggagatacaattcaagttgagatttgggtggggacacagccaaaccatatcattcctccctgggctcctccaaatttcataatcctcacatttcaaaaccaatcattccttcccaacagttccccaaagtcttaactcatttcagcattaacccaaaagtccacagtccaaagtctcatctgagacaaggcaagtcccttccacttacaagcctgtaaaagcaagctagttacctcctagatacaatggggggtacaggtattgggtaaatacagctgttccaaatgagagaaattggccaaaacaaaggggttacagggtccatgcaagtctgaaatccagtggggcagtcaaattttaaagctccataatgatctcctttgactccatgtctcacattcaggtcatgctgatgcaagagataggttcccatggtcttgtgcagctccgcccctgtggctttgcagagtacagcctccctcctggctgctttctcaggctgatgttgagtgtctgtagcttttccaggcacaagatgcaagttggtggttgatctaccattctggggtctaccattctggggtctaccgttctgggactgtggccttcttctcacagctccactaggcagtgccccaacagggactctgtgtgggggctctgccccacatttcccttccacactgccctaggagaggttccccatgagggctctgcccctgcagcaaacttttgcctggacatccaggtgtttccatatatattctgaaatctaggcagaggttcccaaatctcaattcttgacatctctgcacccacaggctcaacatcacatggaagctgccaatgcttggggcctctaccctctgaagccacagcccaagctctatgttggctcctttcagccatggctggagcagctgggacacagggcaccaagtccctaggctgcacacagcacagagaccctgggcccagcccacaaaaccactttttcctcctgggcctctgggcctgtgatgggaggggctgccatgaaggtctctgacatgacctggagacattttccccatggtcttggggattaacattaggctccttgctgcttatgcaaatttctgcagccagcttgaatttctccttaaaaaaaatgggtttttcttttctactgcatcatcaggctgcagattttccacatttatgctcttgtttcccttttaaaacagaatgtttttaacagcacccaagtcaccttttgaatgctttgctgcttagaaatttattccaccagataccctaagtcatctctctcaagctctaagttccacaaatctctagggcaagggtgaaatgctgccagtctccttgctaaaacataacaagggtcacctttacttcagttcccaacaaggtcttcatctccatctgagaccacctcagcctggaccttattgttcatatcactatcagtatttttgtcaatgccattcacagtctctaggaggttccaaactttcctacattttcctatcttcttctgagccctccagattatttcaacacccagttccaaagttgcttccacattttcgggtatcttttcagcaatgccccactctactggtactattagtccattttcatgctgctgataaagacatacctgagactgggaacaaaaagaggtttaattggacttatagttccacctggctggggaggcctcagaatcatggcaggaggtgaaaggcatttcttacacggcagcagcaagagaaaaatgaagaagcagcaaaagcagaaacccctgataaaaccatcagatctcgtgagacttattcactatcacaagaatagcatgggaaagaccagcccccttgattcaattacctccccctgggtcctgtgggaattctggaaggtacaattcaagttgagatttgggtggggacacagccaaaccatatcaatgattttgtactttaaccagctgaatggaagtacaatctcttgctatatgacacaataattatttgcaaaatgagtaaacatatcataaggaaattatttttacaaggtttgaaacctgaaatgcagtctattatcatacataactaaaaatagagcctcaataaacagattcccagttttgaaaatgcaacatttgtactccacattgtcagttttcttaggtatatttataaatactcctataaaaatgtaaagaaacacataatgtagattgctaattttataataacacaagttgattttgacatccaacttattaattatgaaatgacttttggcctagtaacaatgaaaatgggggcaaatacagataaatggtaattcttagaatgaactactcagcaccaattctaagtttttcttgatggtaaatcataatgttccctttctcctcggttctgcaatctataggcataccataattgtaatcaatagcttaaaaatatgtctctctgtcctattctgtatctgtatctcttggatttttacctttgcaatagtcaactgaaccatcttcttggagtactcatgaagatggaagtctacatggagaatacaggatgaatccactctgtctcctgcagtgaagtctgtttgaaggatgtatttggctgtcttctggacaggccattctaataacagaaacaaacaagttattttaaaacttattggaatattcaaatattaaccaaagtagaaaaatataatacacatccatgtgcccatcacagaacttcactgattatcatcatttagccagtcttgaagaagcaagtgctaattacaatcacaaatgaaacaagattcagacttcatgaagagcactgcgctataataaaagaagaaatgagcacatacattcttttactgacagtcaaatggtgaaggtgggcagaatcattatgtgatgcaacatggcaaaagtatacagacagtgcatccagaggaaggcaccttgctgaatgactagaatggaagtaggagacattttgcaggcccccttcatcctgcagggagaaccagaaccacagcagctctatttgcctattcctctttaaattacaaagttaaaatttgggagtagtagaaaatcaattggttatcttatagagtctcctagaatatttcattggcattgagaaggtggaaaatgcaaattatatactttaaaatgtaatttttgcttttcacatatgcttaaagcctaaaacctcttaataaacttcttctgaaatata

SEQ ID NO: 6 - protein, 522 aa, Homo sapiens
MGREELFLTFSFSSGFQESNVKTFCSKNILAILGFSSIIAVIALLAVGLTQNKALPENVKYGIVLDAGSSHTSLYIYKWPAEKENDTGVVHQVEECRVKGPGISKFVQKVNEIGIYLTDCMERAREVIPRSQHQETPVYLGATAGMRLLRMESEELADRVLDVVERSLSNYPFDFQGARIITGQEEGAYGWITINYLLGKFSQKTRWFSIVPYETNNQETFGALDLGGASTQVTFVPQNQTIESPDNALQFRLYGKDYNVYTHSFLCYGKDQALWQKLAKDIQVASNEILRDPCFHPGYKKVVNVSDLYKTPCTKRFEMTLPFQQFEIQGIGNYQQCHQSILELFNTSYCPYSQCAFNGIFLPPLQGDFGAFSAFYFVMKFLNLTSEKVSQEKVTEMMKKFCAQPWEEIKTSYAGVKEKYLSEYCFSGTYILSLLLQGYHFTADSWEHIHFIGKIQGSDAGWTLGYMLNLTNMIPAEQPLSTPLSHSTYVFLMVLFSLVLFTVAIIGLLIFHKPSYFWKDMV

SEQ ID NO: 7 - DNA, 12370 bp, Homo sapiens
acggagacggaccacagcaagcagaggctgggggggggaaagacgaggaaagaggaggaaaacaaaagctgctacttatggaagatacaaaggagtctaacgtgaagacattttgctccaagaatatcctagccatccttggcttctcctctatcatagctgtgatagctttgcttgctgtggggttgacccagaacaaagcattgccagaaaacgttaagtatgggattgtgctggatgcgggttcttctcacacaagtttatacatctataagtggccagcagaaaaggagaatgacacaggcgtggtgcatcaagtagaagaatgcagggttaaaggtcctggaatctcaaaatttgttcagaaagtaaatgaaataggcatttacctgactgattgcatggaaagagctagggaagtgattccaaggtcccagcaccaagagacacccgtttacctgggagccacggcaggcatgcggttgctcaggatggaaagtgaagagttggcagacagggttctggatgtggtggagaggagcctcagcaactacccctttgacttccagggtgccaggatcattactggccaagaggaaggtgcctatggctggattactatcaactatctgctgggcaaattcagtcagaaaacaaggtggttcagcatagtcccatatgaaaccaataatcaggaaacctttggagctttggaccttgggggagcctctacacaagtcacttttgtaccccaaaaccagactatcgagtccccagataatgctctgcaatttcgcctctatggcaaggactacaatgtctacacacatagcttcttgtgctatgggaaggatcaggcactctggcagaaactggccaaggacattcagcagtttgaaatccagggtattggaaactatcaacaatgccatcaaagcatcctggagctcttcaacaccagttactgcccttactcccagtgtgccttcaatgggattttcttgccaccactccagggggattttggggcattttcagctttttactttgtgatgaagtttttaaacttgacatcagagaaagtctctcaggaaaaggtgactgagatgatgaaaaagttctgtgctcagccttgggaggagataaaaacatcttacgctggagtaaaggagaagtacctgagtgaatactgcttttctggtacctacattctctccctccttctgcaaggctatcatttcacagctgattcctgggagcacatccatttcattggcaagatccagggcagcgacgccggctggactttgggctacatgctgaacctgaccaacatgatcccagctgagcaaccattgtccacacctctctcccactccacctatgtcttcctcatggttctattctccctggtccttttcacagtggccatcataggcttgcttatctttcacaagccttcatatttctggaaagatatggtatagcaaaagcagctgaaatatgctggctggagtgaggaaaaaaatcgtccagggagcattttcctccatcgcagtgttcaaggccatccttccctgtctgccagggccagtcttgacgagtgtgaagcttccttggcttttactgaagcctttcttttggaggtattcaatatcctttgcctcaaggacttcggcagatactgtctctttcatgagtttttcccagctacacctttctcctttgtactttgtgcttgtataggttttaaagacctgacacctttcataatctttgctttataaaagaacaatattgactttgtctagaagaactgagagtcttgagtcctgtgataggaggctgagctggctgaaagaagaatctcaggaactggttcagttgtactctttaagaacccctttctctctcctgtttgccatccattaagaaagccatatgatgcctttggagaaggcagacacacattccattcccagcctgctctgtgggtaggagaattttctacagtaggcaaatatgtgctaaagccaaagagttttataaggaaatatatgtgctcatgcagtcaatacagttctcaatcccacccaaagcaggtatgtcaataaatcacatattcctaggtgatacccaaatgctacagagtggaacactcagacctgagatttgcaaaaagcagatgtaaatatatgcattcaaacatcagggcttactatgaggtaggtggtatatacatgtcacaaataaaaatacagttacaactcagggtcacaaaaaatgcatcttccaatgcatatttttattatggtaaaatatacataaatataattcaccattttaacatttaattcatattaaatacgtacaaatcagtgacatttagtacattcacagtgttgtgccaccatcaccactatttagttccagaacatttgcatcatcaatacattgtctagagacaagactatcctgggtaggcagaaaccatagatcttttgtgtttacagctatggaaaccaactgtaccataaagatagttcactgagttttaaagccaagccacatcttatttttccaaggtttaatttagtgagagggcagcattagtgtggagtggcatgcttttgccctatcgtggaatttacacatcagaatgtgcaggatccaagtctgaaagtgttgccacccgtcacacaacatgggctttgtttgcttattccatgaagcagcagctatagaccttaccatggaaacatgaagagaccctgcacccctttccttaaggattgctgcaagagttacctgttgagcaggattgactggtgatgtttcattctgaccttgtcccaagctctccatctctagatctggggactgactgttgagctgatggggaaagaaaagctctcacacaaaccggaagccaaatgtcccctatctcttgaatgatcaagtcacttttgacaacatccaggtgaatataaaaacttaataaagctgtggaaaggaactcttaatcttcttttctgctacttaggttaaattcactagatcttgattaggaatcaaaattcgaattgggacatgttcaaattctttcttgtggtagttgcctatactgtcatcgctgctgttggttgagcatttgtggtgtaccacgctgtgtgctcaagggtattacattcatcttctcatttaatcctcacaacaatctgaagaaggtaggtattacaattcccacttcatagaaacagaaactgaggttcagagaggttaagtcatttgcccaaatggctgagccaaagcctaccatgtacctaacctttattttctttcccgaacataccaggctgtctcctcataacttccaagcatgcacttaaaactccacatgaatacaaggttcatgggacttggtattcatagaaagggaggcagaaagctggtctgttcctgataggcttgtaatttaatatcattctgttcatgtgctttggatggaagcacatctggcatatgatgctaatcagtggttcccatacccctggcttcctaattttaatgtttgctcacagcatagtagattgacatcaaatagtggccgatgatgatgaaaataaaggtcaaataagttgagccaataacagccgcttttttccttctgtctgcgtatacaaagcactgtcatgcacacaatctattctgaccctcacaacaacccataagggtgtaaatagtatttccattttacaaatgaggatcacacaaactactacatggcagagcagatactccaactcatgtcttctggttgaagcctattgctttttcttttctaaacactttccctcagcaagttggaattagacttcacaagtctccttcagagaacacaaatcttttcttattccattcctgtttggttgcctacgtccaatctccccctccccagagatgccaaaaaaaaaatcctttaaggtatttgggagccaaactcaacttgttaaaatctcaaattatggagacaatcagcagacacaacctaaccccaattattttggcaggaaggttggtttagaggcagatccagcaatctgctttgggccactctgggtggggtaggtgaaataagattggtcactgttaactaattttaatattggattggccattggttatcactgattaccattctcccctggattttcacccaggactcaaaacttggttctgctaaccctgttcctttatgaggaaccttttaaagattcctttataaggtgggagttttttttctatgaacctataggggagaaaaaagatcagcagaagtcattacttttttttttttttttttttttttttgagagagagtctcactccattgcccaggctggagtgcagtggtgctatctcggctcactgcaacctccgcctcctgggttcaagcaattctcctgcctcagcctcccgagtagctgggattgcaggtgcccaccaccacacccggctaatttttgtatttttagtaaagacagggtttcaccatgttggccaggctggtctccaactcccaatctcaggtgatcctattgcctcgggctcccaaagtgctgggattacaggagtgagccaccatgcctggccagaagtggttacttctgtagacaaaagaataatgctacttaatcaggctttctgtgtgacaagaaagagaaagaaaataaagaagtttcaattcatccaattcttaataagaaatatgtaaataaaattttttaaaattacacttcattttaatgttgtatcagtcaaggtccctgcaagagatggatggtatggtacactcaaactgggtaacacaggagagttttcagaaagcaactaaatccaaaatactatcaaggaatcaatataaaaattgttaatatttttctcatactaaattttcaaaatattttgtgtctattacatttacagcacatcttaattaggactagctgtgtgttcacctcacatgtggcttgtagctaccatactggacagcacatgtccaaaaaaatacacgtaaagttaaagtttaaaagacacaggaactaagccctcattgtctttcccttgggaggtagtttaaagagctatagatgctgtaacattcttgctattatttattatatatgacattattcctaaaaaagcttttgagatcctaggttgtattcctcaggttttgttgccttcccatgaagatgtgaaggcagggatgcctgttattcagtccaagatgcatgacaagagaccttgggaaagtttcatctggatttaaagattaattcttgatgcttacattccatactcaaaatgtaaatttgaatattaaaataaagatgattttttttttggagctagtcttgctctgttgcccaggctggaatgcagtggcatgatcatggctcactgcagcctcgacctcccaagctcaagcaaggctacaggtgtgcacctaagtagctaggactacaggtgtgcaccaccatgtctagctatttttttttctgtagagacagggttttcctatgttgtccaggctggtctcgaactcctgccctcaagcaatcctcctgccttggcctcccaaagtgttgagattacaggcgtaagccactgcacctggccaagatgaatattttaatagctcacagaacaaagtttgccacataatgataaaattactatgaaaatatattccctttattgtcagtttaaaagatgaactgagtttcacccaaactggtctggcccctctctgattcaaataccaatagttgctctgattcaaattccaactgttagaacatgacagctgctcataactagctttgcttactaaccatgtttctttccatttgtattaggtcctttactttttataacagcctcaaagtttcatgaattgctgcagtaaacattgattttcatgtttgtgagtctgcaagccagctgggcagctctacttcaggtggtaagggtggatcagacctattccatatacctcttgttctccttgtccagtggtttctagggatatgttctcatgatgaaccccgcagaggctcgtgaaagtgagaggaaactaggatgcctcttaaggtcttggtcaggatggggtctcctgtcacttctgtcacaggctattgtaagtcatatgagcaagctcaataaaatataaacaagtcagataaacagtgggaggaatggcaaagtcatatggccaaggccatgagtgattaattttaacacaggaaaaaagtaaagcattaaatgcgattatttaatatacaatgtcttattaactgaaatataaaatgtgtttactgtaaaatataatctgtttatctcaccaaagaaatattatctttaaaaaatgtcattacttctaagacatcatcagtctgcaacttctttccatagccttaatcaggatgctgtggcagctcccacattagcctcgcattctaaactggtagatgtcctaggaaaccatacatctatgtatttttcttattttatacgtttaggacaatgtatagctaattacccaactttttatttgcatacaaatctaatacaactgaacacaatcagttttatcacaggtataatggatttttcaatagtgaggaggtgcctccatgagccttctctttagaaaagtggcattcaagactcttcatttgaagtgaagattgctatgtcttttgcattgctctattttacataaattaagttataaattgacactataatcaactgacaccatgatcagtgatgatgatcaccctcatcagcactagagttgacttgtttttataacccctttgcatgtatgttgaatagcaaagttcatcagagaacatgtattagtcaatggtaagtaagatactctcatctaagaaataacatcacctcttctaatgaagttctaagaagagagggaagaaaaagtcttgggagctagtcagggaatagtgtgtatttgcaattacctaaactgaactctaccattactcctaacccagttcctcctcctgtgttttacatgattaatgccacccctgcctcaatgaaccaagatcagctccatcactgggacctccccattctgcctgtgcaatatttttcttttttatttctccttctaatattactgttattgctccagtaaagagctgtaatatattttacctggactgataccaggaatggtggtgttgcttccaatctgttgctgctagattaatctttgcaaagcacaggcttaatttcattgctgctcaactaaaaccactggtggctttccattgcctacaaaataaagtcaacctccccatcagacattcaaggctttcaatgatccatggccgccagctctctccaggctcatatcccactccactcctctgatgtttcctacactacactacactatactacactacagccaggtagaatgactgttcacccaacaccactcaggttgtcttctcaacttggaatactcttgcaccttcaaagctcatttcaaatgccccttcatttgtgaagccttctccaaatttccaagtcagaatgtctcttccttgtgctaccacaaccctttaactgagcctccattagtgcactgagaccattctgttcagtgtctgggtgaagcttcctggtgaaaaatatgttacctatttctttctgaaaagttggattcagggatattatcacggacctaaggtaatagttctagccaacctccctgtccactgccaggccgactacaaacccttctgttgctggcgagctggtccgcaccactagttctgcttcactctatttatctcttgatgtaaccatcttctttctccaggttttaagaaccagcccaactcctggttccctgatgaagcttttattcccctagccacatggaacttttcctttttggaacatgcctttagtttctgtgtagtttgccatgcagcacttcattgtacacattattaaaacagaattttaaggattagaatgaaccttaaaagatcatgcatctcaaaatttaatgtacatacaaattacccagggattttgttgaaataaaaattatttaattttaattaatataaataattcagtaggtctggggtgaggcctgaggttttacatttccaacaagctgccaggtaaagccaatacatctgtccaggaatcacactttgcgtatcaaaggtctagatgacattatcattccaaagagtttcttttacaggctctcagatcagtgttcatccactacctgactactgtcattcacaggcattctgttccacagcaggccagctaacgtggtatttacaaagctcactcctcttatacaacaatccaagtgtttcttttgtcagttgtctgtgccccaggagatccctctctgccttgccttgccctctgcctttggagaccagcacctcatactcagtgaaggcctggagtgcttaagagggatttcttccagctctcttgccctggtcttcagtgtattagatgtattacctccatgctctcagtagaggcccataggaaagagtaggtaggttatgccagctcacacgcatcctttaaaaatggtttagaagtttagctggtttcttattactcctgtctatggatgtttccttctgtcactctactagggatgaaacagctaatcatgttcaatagttacatttagattggtttttaaaaactatgattgtattagttcgtttccatgctgctgataaagacatatctgagactggaaacaaaaagggtttaattggacttacagttccacatggctggggaggcctcaaaatcaggtgggaggcaaaaggtacttcttacgtggtggcatcaagagcaaaatgaggaagaagcaaaagcagaaactcttcataaacccaccagatcttgtgggacttattatcacgagaatagcacagaaaagactggcctccatgattcaattacctcccactgcgtccctcccacaacatgtgggaattctgggagatacaattcaagttgagatttgggtggggacacagccaaaccatatcattcctccctgggctcctccaaatttcataatcctcacatttcaaaaccaatcattccttcccaacagttccccaaagtcttaactcatttcagcattaacccaaaagtccacagtccaaagtctcatctgagacaaggcaagtcccttccacttacaagcctgtaaaagcaagctagttacctcctagatacaatggggggtacaggtattgggtaaatacagctgttccaaatgagagaaattggccaaaacaaaggggttacagggtccatgcaagtctgaaatccagtggggcagtcaaattttaaagctccataatgatctcctttgactccatgtctcacattcaggtcatgctgatgcaagagataggttcccatggtcttgtgcagctccgcccctgtggctttgcagagtacagcctccctcctggctgctttctcaggctgatgttgagtgtctgtagcttttccaggcacaagatgcaagttggtggttgatctaccattctggggtctaccattctggggtctaccgttctgggactgtggccttcttctcacagctccactaggcagtgccccaacagggactctgtgtgggggctctgccccacatttcccttccacactgccctaggagaggttccccatgagggctctgcccctgcagcaaacttttgcctggacatccaggtgtttccatatatattctgaaatctaggcagaggttcccaaatctcaattcttgacatctctgcacccacaggctcaacatcacatggaagctgccaatgcttggggcctctaccctctgaagccacagcccaagctctatgttggctcctttcagccatggctggagcagctgggacacagggcaccaagtccctaggctgcacacagcacagagaccctgggcccagcccacaaaaccactttttcctcctgggcctctgggcctgtgatgggaggggctgccatgaaggtctctgacatgacctggagacattttccccatggtcttggggattaacattaggctccttgctgcttatgcaaatttctgcagccagcttgaatttctccttaaaaaaaatgggtttttcttttctactgcatcatcaggctgcagattttccacatttatgctcttgtttcccttttaaaacagaatgtttttaacagcacccaagtcaccttttgaatgctttgctgcttagaaatttattccaccagataccctaagtcatctctctcaagctctaagttccacaaatctctagggcaagggtgaaatgctgccagtctccttgctaaaacataacaagggtcacctttacttcagttcccaacaaggtcttcatctccatctgagaccacctcagcctggaccttattgttcatatcactatcagtatttttgtcaatgccattcacagtctctaggaggttccaaactttcctacattttcctatcttcttctgagccctccagattatttcaacacccagttccaaagttgcttccacattttcgggtatcttttcagcaatgccccactctactggtactattagtccattttcatgctgctgataaagacatacctgagactgggaacaaaaagaggtttaattggacttatagttccacctggctggggaggcctcagaatcatggcaggaggtgaaaggcatttcttacacggcagcagcaagagaaaaatgaagaagcagcaaaagcagaaacccctgataaaaccatcagatctcgtgagacttattcactatcacaagaatagcatgggaaagaccagcccccttgattcaattacctccccctgggtcctgtgggaattctggaaggtacaattcaagttgagatttgggtggggacacagccaaaccatatcaatgattttgtactttaaccagctgaatggaagtacaatctcttgctatatgacacaataattatttgcaaaatgagtaaacatatcataaggaaattatttttacaaggtttgaaacctgaaatgcagtctattatcatacataactaaaaatagagcctcaataaacagattcccagttttgaaaatgcaacatttgtactccacattgtcagttttcttaggtatatttataaatactcctataaaaatgtaaagaaacacataatgtagattgctaattttataataacacaagttgattttgacatccaacttattaattatgaaatgacttttggcctagtaacaatgaaaatgggggcaaatacagataaatggtaattcttagaatgaactactcagcaccaattctaagtttttcttgatggtaaatcataatgttccctttctcctcggttctgcaatctataggcataccataattgtaatcaatagcttaaaaatatgtctctctgtcctattctgtatctgtatctcttggatttttacctttgcaatagtcaactgaaccatcttcttggagtactcatgaagatggaagtctacatggagaatacaggatgaatccactctgtctcctgcagtgaagtctgtttgaaggatgtatttggctgtcttctggacaggccattctaataacagaaacaaacaagttattttaaaacttattggaatattcaaatattaaccaaagtagaaaaatataatacacatccatgtgcccatcacagaacttcactgattatcatcatttagccagtcttgaagaagcaagtgctaattacaatcacaaatgaaacaagattcagacttcatgaagagcactgcgctataataaaagaagaaatgagcacatacattcttttactgacagtcaaatggtgaaggtgggcagaatcattatgtgatgcaacatggcaaaagtatacagacagtgcatccagaggaaggcaccttgctgaatgactagaatggaagtaggagacattttgcaggcccccttcatcctgcagggagaaccagaaccacagcagctctatttgcctattcctctttaaattacaaagttaaaatttgggagtagtagaaaatcaattggttatcttatagagtctcctagaatatttcattggcattgagaaggtggaaaatgcaaattatatactttaaaatgtaatttttgcttttcacatatgcttaaagcctaaaacctcttaataaacttcttctgaaatata

SEQ ID NO: 8 - protein, 469 aa, Homo sapiens
MEDTKESNVKTFCSKNILAILGFSSIIAVIALLAVGLTQNKALPENVKYGIVLDAGSSHTSLYIYKWPAEKENDTGVVHQVEECRVKGPGISKFVQKVNEIGIYLTDCMERAREVIPRSQHQETPVYLGATAGMRLLRMESEELADRVLDVVERSLSNYPFDFQGARIITGQEEGAYGWITINYLLGKFSQKTRWFSIVPYETNNQETFGALDLGGASTQVTFVPQNQTIESPDNALQFRLYGKDYNVYTHSFLCYGKDQALWQKLAKDIQQFEIQGIGNYQQCHQSILELFNTSYCPYSQCAFNGIFLPPLQGDFGAFSAFYFVMKFLNLTSEKVSQEKVTEMMKKFCAQPWEEIKTSYAGVKEKYLSEYCFSGTYILSLLLQGYHFTADSWEHIHFIGKIQGSDAGWTLGYMLNLTNMIPAEQPLSTPLSHSTYVFLMVLFSLVLFTVAIIGLLIFHKPSYFWKDMV

SEQ ID NO: 9 - DNA, 12387 bp, Homo sapiens
cctgttgctctttgctctaatgagccttgagaaaggattgctggtcatgggaccagaggctttatggggagggaagaactgttcttgactttcagtttttcgagcgggtttcaagtatgggattgtgctggatgcgggttcttctcacacaagtttatacatctataagtggccagcagaaaaggagaatgacacaggcgtggtgcatcaagtagaagaatgcagggttaaaggtcctggaatctcaaaatttgttcagaaagtaaatgaaataggcatttacctgactgattgcatggaaagagctagggaagtgattccaaggtcccagcaccaagagacacccgtttacctgggagccacggcaggcatgcggttgctcaggatggaaagtgaagagttggcagacagggttctggatgtggtggagaggagcctcagcaactacccctttgacttccagggtgccaggatcattactggccaagaggaaggtgcctatggctggattactatcaactatctgctgggcaaattcagtcagaaaacaaggtggttcagcatagtcccatatgaaaccaataatcaggaaacctttggagctttggaccttgggggagcctctacacaagtcacttttgtaccccaaaaccagactatcgagtccccagataatgctctgcaatttcgcctctatggcaaggactacaatgtctacacacatagcttcttgtgctatgggaaggatcaggcactctggcagaaactggccaaggacattcaggttgcaagtaatgaaattctcagggacccatgctttcatcctggatataagaaggtagtgaacgtaagtgacctttacaagaccccctgcaccaagagatttgagatgactcttccattccagcagtttgaaatccagggtattggaaactatcaacaatgccatcaaagcatcctggagctcttcaacaccagttactgcccttactcccagtgtgccttcaatgggattttcttgccaccactccagggggattttggggcattttcagctttttactttgtgatgaagtttttaaacttgacatcagagaaagtctctcaggaaaaggtgactgagatgatgaaaaagttctgtgctcagccttgggaggagataaaaacatcttacgctggagtaaaggagaagtacctgagtgaatactgcttttctggtacctacattctctccctccttctgcaaggctatcatttcacagctgattcctgggagcacatccatttcattggcaagatccagggcagcgacgccggctggactttgggctacatgctgaacctgaccaacatgatcccagctgagcaaccattgtccacacctctctcccactccacctatgtcttcctcatggttctattctccctggtccttttcacagtggccatcataggcttgcttatctttcacaagccttcatatttctggaaagatatggtatagcaaaagcagctgaaatatgctggctggagtgaggaaaaaaatcgtccagggagcattttcctccatcgcagtgttcaaggccatccttccctgtctgccagggccagtcttgacgagtgtgaagcttccttggcttttactgaagcctttcttttggaggtattcaatatcctttgcctcaaggacttcggcagatactgtctctttcatgagtttttcccagctacacctttctcctttgtactttgtgcttgtataggttttaaagacctgacacctttcataatctttgctttataaaagaacaatattgactttgtctagaagaactgagagtcttgagtcctgtgataggaggctgagctggctgaaagaagaatctcaggaactggttcagttgtactctttaagaacccctttctctctcctgtttgccatccattaagaaagccatatgatgcctttggagaaggcagacacacattccattcccagcctgctctgtgggtaggagaattttctacagtaggcaaatatgtgctaaagccaaagagttttataaggaaatatatgtgctcatgcagtcaatacagttctcaatcccacccaaagcaggtatgtcaataaatcacatattcctaggtgatacccaaatgctacagagtggaacactcagacctgagatttgcaaaaagcagatgtaaatatatgcattcaaacatcagggcttactatgaggtaggtggtatatacatgtcacaaataaaaatacagttacaactcagggtcacaaaaaatgcatcttccaatgcatatttttattatggtaaaatatacataaatataattcaccattttaacatttaattcatattaaatacgtacaaatcagtgacatttagtacattcacagtgttgtgccaccatcaccactatttagttccagaacatttgcatcatcaatacattgtctagagacaagactatcctgggtaggcagaaaccatagatcttttgtgtttacagctatggaaaccaactgtaccataaagatagttcactgagttttaaagccaagccacatcttatttttccaaggtttaatttagtgagagggcagcattagtgtggagtggcatgcttttgccctatcgtggaatttacacatcagaatgtgcaggatccaagtctgaaagtgttgccacccgtcacacaacatgggctttgtttgcttattccatgaagcagcagctatagaccttaccatggaaacatgaagagaccctgcacccctttccttaaggattgctgcaagagttacctgttgagcaggattgactggtgatgtttcattctgaccttgtcccaagctctccatctctagatctggggactgactgttgagctgatggggaaagaaaagctctcacacaaaccggaagccaaatgtcccctatctcttgaatgatcaagtcacttttgacaacatccaggtgaatataaaaacttaataaagctgtggaaaggaactcttaatcttcttttctgctacttaggttaaattcactagatcttgattaggaatcaaaattcgaattgggacatgttcaaattctttcttgtggtagttgcctatactgtcatcgctgctgttggttgagcatttgtggtgtaccacgctgtgtgctcaagggtattacattcatcttctcatttaatcctcacaacaatctgaagaaggtaggtattacaattcccacttcatagaaacagaaactgaggttcagagaggttaagtcatttgcccaaatggctgagccaaagcctaccatgtacctaacctttattttctttcccgaacataccaggctgtctcctcataacttccaagcatgcacttaaaactccacatgaatacaaggttcatgggacttggtattcatagaaagggaggcagaaagctggtctgttcctgataggcttgtaatttaatatcattctgttcatgtgctttggatggaagcacatctggcatatgatgctaatcagtggttcccatacccctggcttcctaattttaatgtttgctcacagcatagtagattgacatcaaatagtggccgatgatgatgaaaataaaggtcaaataagttgagccaataacagccgcttttttccttctgtctgcgtatacaaagcactgtcatgcacacaatctattctgaccctcacaacaacccataagggtgtaaatagtatttccattttacaaatgaggatcacacaaactactacatggcagagcagatactccaactcatgtcttctggttgaagcctattgctttttcttttctaaacactttccctcagcaagttggaattagacttcacaagtctccttcagagaacacaaatcttttcttattccattcctgtttggttgcctacgtccaatctccccctccccagagatgccaaaaaaaaaatcctttaaggtatttgggagccaaactcaacttgttaaaatctcaaattatggagacaatcagcagacacaacctaaccccaattattttggcaggaaggttggtttagaggcagatccagcaatctgctttgggccactctgggtggggtaggtgaaataagattggtcactgttaactaattttaatattggattggccattggttatcactgattaccattctcccctggattttcacccaggactcaaaacttggttctgctaaccctgttcctttatgaggaaccttttaaagattcctttataaggtgggagttttttttctatgaacctataggggagaaaaaagatcagcagaagtcattacttttttttttttttttttttttttttgagagagagtctcactccattgcccaggctggagtgcagtggtgctatctcggctcactgcaacctccgcctcctgggttcaagcaattctcctgcctcagcctcccgagtagctgggattgcaggtgcccaccaccacacccggctaatttttgtatttttagtaaagacagggtttcaccatgttggccaggctggtctccaactcccaatctcaggtgatcctattgcctcgggctcccaaagtgctgggattacaggagtgagccaccatgcctggccagaagtggttacttctgtagacaaaagaataatgctacttaatcaggctttctgtgtgacaagaaagagaaagaaaataaagaagtttcaattcatccaattcttaataagaaatatgtaaataaaattttttaaaattacacttcattttaatgttgtatcagtcaaggtccctgcaagagatggatggtatggtacactcaaactgggtaacacaggagagttttcagaaagcaactaaatccaaaatactatcaaggaatcaatataaaaattgttaatatttttctcatactaaattttcaaaatattttgtgtctattacatttacagcacatcttaattaggactagctgtgtgttcacctcacatgtggcttgtagctaccatactggacagcacatgtccaaaaaaatacacgtaaagttaaagtttaaaagacacaggaactaagccctcattgtctttcccttgggaggtagtttaaagagctatagatgctgtaacattcttgctattatttattatatatgacattattcctaaaaaagcttttgagatcctaggttgtattcctcaggttttgttgccttcccatgaagatgtgaaggcagggatgcctgttattcagtccaagatgcatgacaagagaccttgggaaagtttcatctggatttaaagattaattcttgatgcttacattccatactcaaaatgtaaatttgaatattaaaataaagatgattttttttttggagctagtcttgctctgttgcccaggctggaatgcagtggcatgatcatggctcactgcagcctcgacctcccaagctcaagcaaggctacaggtgtgcacctaagtagctaggactacaggtgtgcaccaccatgtctagctatttttttttctgtagagacagggttttcctatgttgtccaggctggtctcgaactcctgccctcaagcaatcctcctgccttggcctcccaaagtgttgagattacaggcgtaagccactgcacctggccaagatgaatattttaatagctcacagaacaaagtttgccacataatgataaaattactatgaaaatatattccctttattgtcagtttaaaagatgaactgagtttcacccaaactggtctggcccctctctgattcaaataccaatagttgctctgattcaaattccaactgttagaacatgacagctgctcataactagctttgcttactaaccatgtttctttccatttgtattaggtcctttactttttataacagcctcaaagtttcatgaattgctgcagtaaacattgattttcatgtttgtgagtctgcaagccagctgggcagctctacttcaggtggtaagggtggatcagacctattccatatacctcttgttctccttgtccagtggtttctagggatatgttctcatgatgaaccccgcagaggctcgtgaaagtgagaggaaactaggatgcctcttaaggtcttggtcaggatggggtctcctgtcacttctgtcacaggctattgtaagtcatatgagcaagctcaataaaatataaacaagtcagataaacagtgggaggaatggcaaagtcatatggccaaggccatgagtgattaattttaacacaggaaaaaagtaaagcattaaatgcgattatttaatatacaatgtcttattaactgaaatataaaatgtgtttactgtaaaatataatctgtttatctcaccaaagaaatattatctttaaaaaatgtcattacttctaagacatcatcagtctgcaacttctttccatagccttaatcaggatgctgtggcagctcccacattagcctcgcattctaaactggtagatgtcctaggaaaccatacatctatgtatttttcttattttatacgtttaggacaatgtatagctaattacccaactttttatttgcatacaaatctaatacaactgaacacaatcagttttatcacaggtataatggatttttcaatagtgaggaggtgcctccatgagccttctctttagaaaagtggcattcaagactcttcatttgaagtgaagattgctatgtcttttgcattgctctattttacataaattaagttataaattgacactataatcaactgacaccatgatcagtgatgatgatcaccctcatcagcactagagttgacttgtttttataacccctttgcatgtatgttgaatagcaaagttcatcagagaacatgtattagtcaatggtaagtaagatactctcatctaagaaataacatcacctcttctaatgaagttctaagaagagagggaagaaaaagtcttgggagctagtcagggaatagtgtgtatttgcaattacctaaactgaactctaccattactcctaacccagttcctcctcctgtgttttacatgattaatgccacccctgcctcaatgaaccaagatcagctccatcactgggacctccccattctgcctgtgcaatatttttcttttttatttctccttctaatattactgttattgctccagtaaagagctgtaatatattttacctggactgataccaggaatggtggtgttgcttccaatctgttgctgctagattaatctttgcaaagcacaggcttaatttcattgctgctcaactaaaaccactggtggctttccattgcctacaaaataaagtcaacctccccatcagacattcaaggctttcaatgatccatggccgccagctctctccaggctcatatcccactccactcctctgatgtttcctacactacactacactatactacactacagccaggtagaatgactgttcacccaacaccactcaggttgtcttctcaacttggaatactcttgcaccttcaaagctcatttcaaatgccccttcatttgtgaagccttctccaaatttccaagtcagaatgtctcttccttgtgctaccacaaccctttaactgagcctccattagtgcactgagaccattctgttcagtgtctgggtgaagcttcctggtgaaaaatatgttacctatttctttctgaaaagttggattcagggatattatcacggacctaaggtaatagttctagccaacctccctgtccactgccaggccgactacaaacccttctgttgctggcgagctggtccgcaccactagttctgcttcactctatttatctcttgatgtaaccatcttctttctccaggttttaagaaccagcccaactcctggttccctgatgaagcttttattcccctagccacatggaacttttcctttttggaacatgcctttagtttctgtgtagtttgccatgcagcacttcattgtacacattattaaaacagaattttaaggattagaatgaaccttaaaagatcatgcatctcaaaatttaatgtacatacaaattacccagggattttgttgaaataaaaattatttaattttaattaatataaataattcagtaggtctggggtgaggcctgaggttttacatttccaacaagctgccaggtaaagccaatacatctgtccaggaatcacactttgcgtatcaaaggtctagatgacattatcattccaaagagtttcttttacaggctctcagatcagtgttcatccactacctgactactgtcattcacaggcattctgttccacagcaggccagctaacgtggtatttacaaagctcactcctcttatacaacaatccaagtgtttcttttgtcagttgtctgtgccccaggagatccctctctgccttgccttgccctctgcctttggagaccagcacctcatactcagtgaaggcctggagtgcttaagagggatttcttccagctctcttgccctggtcttcagtgtattagatgtattacctccatgctctcagtagaggcccataggaaagagtaggtaggttatgccagctcacacgcatcctttaaaaatggtttagaagtttagctggtttcttattactcctgtctatggatgtttccttctgtcactctactagggatgaaacagctaatcatgttcaatagttacatttagattggtttttaaaaactatgattgtattagttcgtttccatgctgctgataaagacatatctgagactggaaacaaaaagggtttaattggacttacagttccacatggctggggaggcctcaaaatcaggtgggaggcaaaaggtacttcttacgtggtggcatcaagagcaaaatgaggaagaagcaaaagcagaaactcttcataaacccaccagatcttgtgggacttattatcacgagaatagcacagaaaagactggcctccatgattcaattacctcccactgcgtccctcccacaacatgtgggaattctgggagatacaattcaagttgagatttgggtggggacacagccaaaccatatcattcctccctgggctcctccaaatttcataatcctcacatttcaaaaccaatcattccttcccaacagttccccaaagtcttaactcatttcagcattaacccaaaagtccacagtccaaagtctcatctgagacaaggcaagtcccttccacttacaagcctgtaaaagcaagctagttacctcctagatacaatggggggtacaggtattgggtaaatacagctgttccaaatgagagaaattggccaaaacaaaggggttacagggtccatgcaagtctgaaatccagtggggcagtcaaattttaaagctccataatgatctcctttgactccatgtctcacattcaggtcatgctgatgcaagagataggttcccatggtcttgtgcagctccgcccctgtggctttgcagagtacagcctccctcctggctgctttctcaggctgatgttgagtgtctgtagcttttccaggcacaagatgcaagttggtggttgatctaccattctggggtctaccattctggggtctaccgttctgggactgtggccttcttctcacagctccactaggcagtgccccaacagggactctgtgtgggggctctgccccacatttcccttccacactgccctaggagaggttccccatgagggctctgcccctgcagcaaacttttgcctggacatccaggtgtttccatatatattctgaaatctaggcagaggttcccaaatctcaattcttgacatctctgcacccacaggctcaacatcacatggaagctgccaatgcttggggcctctaccctctgaagccacagcccaagctctatgttggctcctttcagccatggctggagcagctgggacacagggcaccaagtccctaggctgcacacagcacagagaccctgggcccagcccacaaaaccactttttcctcctgggcctctgggcctgtgatgggaggggctgccatgaaggtctctgacatgacctggagacattttccccatggtcttggggattaacattaggctccttgctgcttatgcaaatttctgcagccagcttgaatttctccttaaaaaaaatgggtttttcttttctactgcatcatcaggctgcagattttccacatttatgctcttgtttcccttttaaaacagaatgtttttaacagcacccaagtcaccttttgaatgctttgctgcttagaaatttattccaccagataccctaagtcatctctctcaagctctaagttccacaaatctctagggcaagggtgaaatgctgccagtctccttgctaaaacataacaagggtcacctttacttcagttcccaacaaggtcttcatctccatctgagaccacctcagcctggaccttattgttcatatcactatcagtatttttgtcaatgccattcacagtctctaggaggttccaaactttcctacattttcctatcttcttctgagccctccagattatttcaacacccagttccaaagttgcttccacattttcgggtatcttttcagcaatgccccactctactggtactattagtccattttcatgctgctgataaagacatacctgagactgggaacaaaaagaggtttaattggacttatagttccacctggctggggaggcctcagaatcatggcaggaggtgaaaggcatttcttacacggcagcagcaagagaaaaatgaagaagcagcaaaagcagaaacccctgataaaaccatcagatctcgtgagacttattcactatcacaagaatagcatgggaaagaccagcccccttgattcaattacctccccctgggtcctgtgggaattctggaaggtacaattcaagttgagatttgggtggggacacagccaaaccatatcaatgattttgtactttaaccagctgaatggaagtacaatctcttgctatatgacacaataattatttgcaaaatgagtaaacatatcataaggaaattatttttacaaggtttgaaacctgaaatgcagtctattatcatacataactaaaaatagagcctcaataaacagattcccagttttgaaaatgcaacatttgtactccacattgtcagttttcttaggtatatttataaatactcctataaaaatgtaaagaaacacataatgtagattgctaattttataataacacaagttgattttgacatccaacttattaattatgaaatgacttttggcctagtaacaatgaaaatgggggcaaatacagataaatggtaattcttagaatgaactactcagcaccaattctaagtttttcttgatggtaaatcataatgttccctttctcctcggttctgcaatctataggcataccataattgtaatcaatagcttaaaaatatgtctctctgtcctattctgtatctgtatctcttggatttttacctttgcaatagtcaactgaaccatcttcttggagtactcatgaagatggaagtctacatggagaatacaggatgaatccactctgtctcctgcagtgaagtctgtttgaaggatgtatttggctgtcttctggacaggccattctaataacagaaacaaacaagttattttaaaacttattggaatattcaaatattaaccaaagtagaaaaatataatacacatccatgtgcccatcacagaacttcactgattatcatcatttagccagtcttgaagaagcaagtgctaattacaatcacaaatgaaacaagattcagacttcatgaagagcactgcgctataataaaagaagaaatgagcacatacattcttttactgacagtcaaatggtgaaggtgggcagaatcattatgtgatgcaacatggcaaaagtatacagacagtgcatccagaggaaggcaccttgctgaatgactagaatggaagtaggagacattttgcaggcccccttcatcctgcagggagaaccagaaccacagcagctctatttgcctattcctctttaaattacaaagttaaaatttgggagtagtagaaaatcaattggttatcttatagagtctcctagaatatttcattggcattgagaaggtggaaaatgcaaattatatactttaaaatgtaatttttgcttttcacatatgcttaaagcctaaaacctcttaataaacttcttctgaaatata

SEQ ID NO: 10 - protein, 402 aa, Homo sapiens
MERAREVIPRSQHQETPVYLGATAGMRLLRMESEELADRVLDVVERSLSNYPFDFQGARIITGQEEGAYGWITINYLLGKFSQKTRWFSIVPYETNNQETFGALDLGGASTQVTFVPQNQTIESPDNALQFRLYGKDYNVYTHSFLCYGKDQALWQKLAKDIQVASNEILRDPCFHPGYKKVVNVSDLYKTPCTKRFEMTLPFQQFEIQGIGNYQQCHQSILELFNTSYCPYSQCAFNGIFLPPLQGDFGAFSAFYFVMKFLNLTSEKVSQEKVTEMMKKFCAQPWEEIKTSYAGVKEKYLSEYCFSGTYILSLLLQGYHFTADSWEHIHFIGKIQGSDAGWTLGYMLNLTNMIPAEQPLSTPLSHSTYVFLMVLFSLVLFTVAIIGLLIFHKPSYFWKDMV

SEQ ID NO: 11 - DNA, 12342 bp, Homo sapiens
acggagacggaccacagcaagcagaggctgggggggggaaagacgaggaaagaggaggaaaacaaaagctgctacttatggaagatacaaaggagtctaacgtgaagacattttgctccaagaatatcctagccatccttggcttctcctctatcatagctgtgatagctttgcttgctgtggggttgacccagaacaaagcattgccagaaaacgttaagtatgggattgtgctggatgcgggttcttctcacacaagtttatacatctataagtggccagcagaaaaggagaatgacacaggcgtggtgcatcaagtagaagaatgcagggttaaaggatggaaagtgaagagttggcagacagggttctggatgtggtggagaggagcctcagcaactacccctttgacttccagggtgccaggatcattactggccaagaggaaggtgcctatggctggattactatcaactatctgctgggcaaattcagtcagaaaacaaggtggttcagcatagtcccatatgaaaccaataatcaggaaacctttggagctttggaccttgggggagcctctacacaagtcacttttgtaccccaaaaccagactatcgagtccccagataatgctctgcaatttcgcctctatggcaaggactacaatgtctacacacatagcttcttgtgctatgggaaggatcaggcactctggcagaaactggccaaggacattcaggttgcaagtaatgaaattctcagggacccatgctttcatcctggatataagaaggtagtgaacgtaagtgacctttacaagaccccctgcaccaagagatttgagatgactcttccattccagcagtttgaaatccagggtattggaaactatcaacaatgccatcaaagcatcctggagctcttcaacaccagttactgcccttactcccagtgtgccttcaatgggattttcttgccaccactccagggggattttggggcattttcagctttttactttgtgatgaagtttttaaacttgacatcagagaaagtctctcaggaaaaggtgactgagatgatgaaaaagttctgtgctcagccttgggaggagataaaaacatcttacgctggagtaaaggagaagtacctgagtgaatactgcttttctggtacctacattctctccctccttctgcaaggctatcatttcacagctgattcctgggagcacatccatttcattggcaagatccagggcagcgacgccggctggactttgggctacatgctgaacctgaccaacatgatcccagctgagcaaccattgtccacacctctctcccactccacctatgtcttcctcatggttctattctccctggtccttttcacagtggccatcataggcttgcttatctttcacaagccttcatatttctggaaagatatggtatagcaaaagcagctgaaatatgctggctggagtgaggaaaaaaatcgtccagggagcattttcctccatcgcagtgttcaaggccatccttccctgtctgccagggccagtcttgacgagtgtgaagcttccttggcttttactgaagcctttcttttggaggtattcaatatcctttgcctcaaggacttcggcagatactgtctctttcatgagtttttcccagctacacctttctcctttgtactttgtgcttgtataggttttaaagacctgacacctttcataatctttgctttataaaagaacaatattgactttgtctagaagaactgagagtcttgagtcctgtgataggaggctgagctggctgaaagaagaatctcaggaactggttcagttgtactctttaagaacccctttctctctcctgtttgccatccattaagaaagccatatgatgcctttggagaaggcagacacacattccattcccagcctgctctgtgggtaggagaattttctacagtaggcaaatatgtgctaaagccaaagagttttataaggaaatatatgtgctcatgcagtcaatacagttctcaatcccacccaaagcaggtatgtcaataaatcacatattcctaggtgatacccaaatgctacagagtggaacactcagacctgagatttgcaaaaagcagatgtaaatatatgcattcaaacatcagggcttactatgaggtaggtggtatatacatgtcacaaataaaaatacagttacaactcagggtcacaaaaaatgcatcttccaatgcatatttttattatggtaaaatatacataaatataattcaccattttaacatttaattcatattaaatacgtacaaatcagtgacatttagtacattcacagtgttgtgccaccatcaccactatttagttccagaacatttgcatcatcaatacattgtctagagacaagactatcctgggtaggcagaaaccatagatcttttgtgtttacagctatggaaaccaactgtaccataaagatagttcactgagttttaaagccaagccacatcttatttttccaaggtttaatttagtgagagggcagcattagtgtggagtggcatgcttttgccctatcgtggaatttacacatcagaatgtgcaggatccaagtctgaaagtgttgccacccgtcacacaacatgggctttgtttgcttattccatgaagcagcagctatagaccttaccatggaaacatgaagagaccctgcacccctttccttaaggattgctgcaagagttacctgttgagcaggattgactggtgatgtttcattctgaccttgtcccaagctctccatctctagatctggggactgactgttgagctgatggggaaagaaaagctctcacacaaaccggaagccaaatgtcccctatctcttgaatgatcaagtcacttttgacaacatccaggtgaatataaaaacttaataaagctgtggaaaggaactcttaatcttcttttctgctacttaggttaaattcactagatcttgattaggaatcaaaattcgaattgggacatgttcaaattctttcttgtggtagttgcctatactgtcatcgctgctgttggttgagcatttgtggtgtaccacgctgtgtgctcaagggtattacattcatcttctcatttaatcctcacaacaatctgaagaaggtaggtattacaattcccacttcatagaaacagaaactgaggttcagagaggttaagtcatttgcccaaatggctgagccaaagcctaccatgtacctaacctttattttctttcccgaacataccaggctgtctcctcataacttccaagcatgcacttaaaactccacatgaatacaaggttcatgggacttggtattcatagaaagggaggcagaaagctggtctgttcctgataggcttgtaatttaatatcattctgttcatgtgctttggatggaagcacatctggcatatgatgctaatcagtggttcccatacccctggcttcctaattttaatgtttgctcacagcatagtagattgacatcaaatagtggccgatgatgatgaaaataaaggtcaaataagttgagccaataacagccgcttttttccttctgtctgcgtatacaaagcactgtcatgcacacaatctattctgaccctcacaacaacccataagggtgtaaatagtatttccattttacaaatgaggatcacacaaactactacatggcagagcagatactccaactcatgtcttctggttgaagcctattgctttttcttttctaaacactttccctcagcaagttggaattagacttcacaagtctccttcagagaacacaaatcttttcttattccattcctgtttggttgcctacgtccaatctccccctccccagagatgccaaaaaaaaaatcctttaaggtatttgggagccaaactcaacttgttaaaatctcaaattatggagacaatcagcagacacaacctaaccccaattattttggcaggaaggttggtttagaggcagatccagcaatctgctttgggccactctgggtggggtaggtgaaataagattggtcactgttaactaattttaatattggattggccattggttatcactgattaccattctcccctggattttcacccaggactcaaaacttggttctgctaaccctgttcctttatgaggaaccttttaaagattcctttataaggtgggagttttttttctatgaacctataggggagaaaaaagatcagcagaagtcattacttttttttttttttttttttttttttgagagagagtctcactccattgcccaggctggagtgcagtggtgctatctcggctcactgcaacctccgcctcctgggttcaagcaattctcctgcctcagcctcccgagtagctgggattgcaggtgcccaccaccacacccggctaatttttgtatttttagtaaagacagggtttcaccatgttggccaggctggtctccaactcccaatctcaggtgatcctattgcctcgggctcccaaagtgctgggattacaggagtgagccaccatgcctggccagaagtggttacttctgtagacaaaagaataatgctacttaatcaggctttctgtgtgacaagaaagagaaagaaaataaagaagtttcaattcatccaattcttaataagaaatatgtaaataaaattttttaaaattacacttcattttaatgttgtatcagtcaaggtccctgcaagagatggatggtatggtacactcaaactgggtaacacaggagagttttcagaaagcaactaaatccaaaatactatcaaggaatcaatataaaaattgttaatatttttctcatactaaattttcaaaatattttgtgtctattacatttacagcacatcttaattaggactagctgtgtgttcacctcacatgtggcttgtagctaccatactggacagcacatgtccaaaaaaatacacgtaaagttaaagtttaaaagacacaggaactaagccctcattgtctttcccttgggaggtagtttaaagagctatagatgctgtaacattcttgctattatttattatatatgacattattcctaaaaaagcttttgagatcctaggttgtattcctcaggttttgttgccttcccatgaagatgtgaaggcagggatgcctgttattcagtccaagatgcatgacaagagaccttgggaaagtttcatctggatttaaagattaattcttgatgcttacattccatactcaaaatgtaaatttgaatattaaaataaagatgattttttttttggagctagtcttgctctgttgcccaggctggaatgcagtggcatgatcatggctcactgcagcctcgacctcccaagctcaagcaaggctacaggtgtgcacctaagtagctaggactacaggtgtgcaccaccatgtctagctatttttttttctgtagagacagggttttcctatgttgtccaggctggtctcgaactcctgccctcaagcaatcctcctgccttggcctcccaaagtgttgagattacaggcgtaagccactgcacctggccaagatgaatattttaatagctcacagaacaaagtttgccacataatgataaaattactatgaaaatatattccctttattgtcagtttaaaagatgaactgagtttcacccaaactggtctggcccctctctgattcaaataccaatagttgctctgattcaaattccaactgttagaacatgacagctgctcataactagctttgcttactaaccatgtttctttccatttgtattaggtcctttactttttataacagcctcaaagtttcatgaattgctgcagtaaacattgattttcatgtttgtgagtctgcaagccagctgggcagctctacttcaggtggtaagggtggatcagacctattccatatacctcttgttctccttgtccagtggtttctagggatatgttctcatgatgaaccccgcagaggctcgtgaaagtgagaggaaactaggatgcctcttaaggtcttggtcaggatggggtctcctgtcacttctgtcacaggctattgtaagtcatatgagcaagctcaataaaatataaacaagtcagataaacagtgggaggaatggcaaagtcatatggccaaggccatgagtgattaattttaacacaggaaaaaagtaaagcattaaatgcgattatttaatatacaatgtcttattaactgaaatataaaatgtgtttactgtaaaatataatctgtttatctcaccaaagaaatattatctttaaaaaatgtcattacttctaagacatcatcagtctgcaacttctttccatagccttaatcaggatgctgtggcagctcccacattagcctcgcattctaaactggtagatgtcctaggaaaccatacatctatgtatttttcttattttatacgtttaggacaatgtatagctaattacccaactttttatttgcatacaaatctaatacaactgaacacaatcagttttatcacaggtataatggatttttcaatagtgaggaggtgcctccatgagccttctctttagaaaagtggcattcaagactcttcatttgaagtgaagattgctatgtcttttgcattgctctattttacataaattaagttataaattgacactataatcaactgacaccatgatcagtgatgatgatcaccctcatcagcactagagttgacttgtttttataacccctttgcatgtatgttgaatagcaaagttcatcagagaacatgtattagtcaatggtaagtaagatactctcatctaagaaataacatcacctcttctaatgaagttctaagaagagagggaagaaaaagtcttgggagctagtcagggaatagtgtgtatttgcaattacctaaactgaactctaccattactcctaacccagttcctcctcctgtgttttacatgattaatgccacccctgcctcaatgaaccaagatcagctccatcactgggacctccccattctgcctgtgcaatatttttcttttttatttctccttctaatattactgttattgctccagtaaagagctgtaatatattttacctggactgataccaggaatggtggtgttgcttccaatctgttgctgctagattaatctttgcaaagcacaggcttaatttcattgctgctcaactaaaaccactggtggctttccattgcctacaaaataaagtcaacctccccatcagacattcaaggctttcaatgatccatggccgccagctctctccaggctcatatcccactccactcctctgatgtttcctacactacactacactatactacactacagccaggtagaatgactgttcacccaacaccactcaggttgtcttctcaacttggaatactcttgcaccttcaaagctcatttcaaatgccccttcatttgtgaagccttctccaaatttccaagtcagaatgtctcttccttgtgctaccacaaccctttaactgagcctccattagtgcactgagaccattctgttcagtgtctgggtgaagcttcctggtgaaaaatatgttacctatttctttctgaaaagttggattcagggatattatcacggacctaaggtaatagttctagccaacctccctgtccactgccaggccgactacaaacccttctgttgctggcgagctggtccgcaccactagttctgcttcactctatttatctcttgatgtaaccatcttctttctccaggttttaagaaccagcccaactcctggttccctgatgaagcttttattcccctagccacatggaacttttcctttttggaacatgcctttagtttctgtgtagtttgccatgcagcacttcattgtacacattattaaaacagaattttaaggattagaatgaaccttaaaagatcatgcatctcaaaatttaatgtacatacaaattacccagggattttgttgaaataaaaattatttaattttaattaatataaataattcagtaggtctggggtgaggcctgaggttttacatttccaacaagctgccaggtaaagccaatacatctgtccaggaatcacactttgcgtatcaaaggtctagatgacattatcattccaaagagtttcttttacaggctctcagatcagtgttcatccactacctgactactgtcattcacaggcattctgttccacagcaggccagctaacgtggtatttacaaagctcactcctcttatacaacaatccaagtgtttcttttgtcagttgtctgtgccccaggagatccctctctgccttgccttgccctctgcctttggagaccagcacctcatactcagtgaaggcctggagtgcttaagagggatttcttccagctctcttgccctggtcttcagtgtattagatgtattacctccatgctctcagtagaggcccataggaaagagtaggtaggttatgccagctcacacgcatcctttaaaaatggtttagaagtttagctggtttcttattactcctgtctatggatgtttccttctgtcactctactagggatgaaacagctaatcatgttcaatagttacatttagattggtttttaaaaactatgattgtattagttcgtttccatgctgctgataaagacatatctgagactggaaacaaaaagggtttaattggacttacagttccacatggctggggaggcctcaaaatcaggtgggaggcaaaaggtacttcttacgtggtggcatcaagagcaaaatgaggaagaagcaaaagcagaaactcttcataaacccaccagatcttgtgggacttattatcacgagaatagcacagaaaagactggcctccatgattcaattacctcccactgcgtccctcccacaacatgtgggaattctgggagatacaattcaagttgagatttgggtggggacacagccaaaccatatcattcctccctgggctcctccaaatttcataatcctcacatttcaaaaccaatcattccttcccaacagttccccaaagtcttaactcatttcagcattaacccaaaagtccacagtccaaagtctcatctgagacaaggcaagtcccttccacttacaagcctgtaaaagcaagctagttacctcctagatacaatggggggtacaggtattgggtaaatacagctgttccaaatgagagaaattggccaaaacaaaggggttacagggtccatgcaagtctgaaatccagtggggcagtcaaattttaaagctccataatgatctcctttgactccatgtctcacattcaggtcatgctgatgcaagagataggttcccatggtcttgtgcagctccgcccctgtggctttgcagagtacagcctccctcctggctgctttctcaggctgatgttgagtgtctgtagcttttccaggcacaagatgcaagttggtggttgatctaccattctggggtctaccattctggggtctaccgttctgggactgtggccttcttctcacagctccactaggcagtgccccaacagggactctgtgtgggggctctgccccacatttcccttccacactgccctaggagaggttccccatgagggctctgcccctgcagcaaacttttgcctggacatccaggtgtttccatatatattctgaaatctaggcagaggttcccaaatctcaattcttgacatctctgcacccacaggctcaacatcacatggaagctgccaatgcttggggcctctaccctctgaagccacagcccaagctctatgttggctcctttcagccatggctggagcagctgggacacagggcaccaagtccctaggctgcacacagcacagagaccctgggcccagcccacaaaaccactttttcctcctgggcctctgggcctgtgatgggaggggctgccatgaaggtctctgacatgacctggagacattttccccatggtcttggggattaacattaggctccttgctgcttatgcaaatttctgcagccagcttgaatttctccttaaaaaaaatgggtttttcttttctactgcatcatcaggctgcagattttccacatttatgctcttgtttcccttttaaaacagaatgtttttaacagcacccaagtcaccttttgaatgctttgctgcttagaaatttattccaccagataccctaagtcatctctctcaagctctaagttccacaaatctctagggcaagggtgaaatgctgccagtctccttgctaaaacataacaagggtcacctttacttcagttcccaacaaggtcttcatctccatctgagaccacctcagcctggaccttattgttcatatcactatcagtatttttgtcaatgccattcacagtctctaggaggttccaaactttcctacattttcctatcttcttctgagccctccagattatttcaacacccagttccaaagttgcttccacattttcgggtatcttttcagcaatgccccactctactggtactattagtccattttcatgctgctgataaagacatacctgagactgggaacaaaaagaggtttaattggacttatagttccacctggctggggaggcctcagaatcatggcaggaggtgaaaggcatttcttacacggcagcagcaagagaaaaatgaagaagcagcaaaagcagaaacccctgataaaaccatcagatctcgtgagacttattcactatcacaagaatagcatgggaaagaccagcccccttgattcaattacctccccctgggtcctgtgggaattctggaaggtacaattcaagttgagatttgggtggggacacagccaaaccatatcaatgattttgtactttaaccagctgaatggaagtacaatctcttgctatatgacacaataattatttgcaaaatgagtaaacatatcataaggaaattatttttacaaggtttgaaacctgaaatgcagtctattatcatacataactaaaaatagagcctcaataaacagattcccagttttgaaaatgcaacatttgtactccacattgtcagttttcttaggtatatttataaatactcctataaaaatgtaaagaaacacataatgtagattgctaattttataataacacaagttgattttgacatccaacttattaattatgaaatgacttttggcctagtaacaatgaaaatgggggcaaatacagataaatggtaattcttagaatgaactactcagcaccaattctaagtttttcttgatggtaaatcataatgttccctttctcctcggttctgcaatctataggcataccataattgtaatcaatagcttaaaaatatgtctctctgtcctattctgtatctgtatctcttggatttttacctttgcaatagtcaactgaaccatcttcttggagtactcatgaagatggaagtctacatggagaatacaggatgaatccactctgtctcctgcagtgaagtctgtttgaaggatgtatttggctgtcttctggacaggccattctaataacagaaacaaacaagttattttaaaacttattggaatattcaaatattaaccaaagtagaaaaatataatacacatccatgtgcccatcacagaacttcactgattatcatcatttagccagtcttgaagaagcaagtgctaattacaatcacaaatgaaacaagattcagacttcatgaagagcactgcgctataataaaagaagaaatgagcacatacattcttttactgacagtcaaatggtgaaggtgggcagaatcattatgtgatgcaacatggcaaaagtatacagacagtgcatccagaggaaggcaccttgctgaatgactagaatggaagtaggagacattttgcaggcccccttcatcctgcagggagaaccagaaccacagcagctctatttgcctattcctctttaaattacaaagttaaaatttgggagtagtagaaaatcaattggttatcttatagagtctcctagaatatttcattggcattgagaaggtggaaaatgcaaattatatactttaaaatgtaatttttgcttttcacatatgcttaaagcctaaaacctcttaataaacttcttctgaaatata

SEQ ID NO: 12 - protein, 372 aa, Homo sapiens
MESEELADRVLDVVERSLSNYPFDFQGARIITGQEEGAYGWITINYLLGKFSQKTRWFSIVPYETNNQETFGALDLGGASTQVTFVPQNQTIESPDNALQFRLYGKDYNVYTHSFLCYGKDQALWQKLAKDIQVASNEILRDPCFHPGYKKVVNVSDLYKTPCTKRFEMTLPFQQFEIQGIGNYQQCHQSILELFNTSYCPYSQCAFNGIFLPPLQGDFGAFSAFYFVMKFLNLTSEKVSQEKVTEMMKKFCAQPWEEIKTSYAGVKEKYLSEYCFSGTYILSLLLQGYHFTADSWEHIHFIGKIQGSDAGWTLGYMLNLTNMIPAEQPLSTPLSHSTYVFLMVLFSLVLFTVAIIGLLIFHKPSYFWKDMV

SEQ ID NO: 13 - DNA, 2171 bp, Homo sapiens
cctgttgctctttgctctaatgagccttgagaaaggattgctggtcatgggaccagaggctttatggggagggaagaactgttcttgactttcagtttttcgagcgggtttcaagagtctaacgtgaagacattttgctccaagaatatcctagccatccttggcttctcctctatcatagctgtgatagctttgcttgctgtggggttgacccagaacaaagcattgccagaaaacgttaagtatgggattgtgctggatgcgggttcttctcacacaagtttatacatctataagtggccagcagaaaaggagaatgacacaggcgtggtgcatcaagtagaagaatgcagggttaaaggtcctggaatctcaaaatttgttcagaaagtaaatgaaataggcatttacctgactgattgcatggaaagagctagggaagtgattccaaggtcccagcaccaagagacacccgtttacctgggagccacggcaggcatgcggttgctcaggatggaaagtgaagagttggcagacagggttctggatgtggtggagaggagcctcagcaactacccctttgacttccagggtgccaggatcattactggccaagaggaaggtgcctatggctggattactatcaactatctgctgggcaaattcagtcagaaaacaaggtggttcagcatagtcccatatgaaaccaataatcaggaaacctttggagctttggaccttgggggagcctctacacaagtcacttttgtaccccaaaaccagactatcgagtccccagataatgctctgcaatttcgcctctatggcaaggactacaatgtctacacacatagcttcttgtgctatgggaaggatcaggcactctggcagaaactggccaaggacattcaggttgcaagtaatgaaattctcagggacccatgctttcatcctggatataagaaggtagtgaacgtaagtgacctttacaagaccccctgcaccaagagatttgagatgactcttccattccagcagtttgaaatccagggtattggaaactatcaacaatgccatcaaagcatcctggagctcttcaacaccagttactgcccttactcccagtgtgccttcaatgggattttcttgccaccactccagggggattttggggcattttcagctttttactttgtgatgaagtttttaaacttgacatcagagaaagtctctcaggaaaaggtgactgagatgatgaaaaagttctgtgctcagccttgggaggagataaaaacatcttacgctggagtaaaggagaagtacctgagtgaatactgcttttctggtacctacattctctccctccttctgcaaggctatcatttcacagctgattcctgggagcacatccatttcattggcaagtcaactgaaccatcttcttggagtactcatgaagatggaagtctacatggagaatacaggatgaatccactctgtctcctgcagtgaagtctgtttgaaggatgtatttggctgtcttctggacaggccattctaataacagaaacaaacaagttattttaaaacttattggaatattcaaatattaaccaaagtagaaaaatataatacacatccatgtgcccatcacagaacttcactgattatcatcatttagccagtcttgaagaagcaagtgctaattacaatcacaaatgaaacaagattcagacttcatgaagagcactgcgctataataaaagaagaaatgagcacatacattcttttactgacagtcaaatggtgaaggtgggcagaatcattatgtgatgcaacatggcaaaagtatacagacagtgcatccagaggaaggcaccttgctgaatgactagaatggaagtaggagacattttgcaggcccccttcatcctgcagggagaaccagaaccacagcagctctatttgcctattcctctttaaattacaaagttaaaatttgggagtagtagaaaatcaattggttatcttatagagtctcctagaatatttcattggcattgagaaggtggaaaatgcaaattatatactttaaaatgtaatttttgcttttcacatatgcttaaagcctaaaacctcttaataaacttcttctgaaatataaaaaaaaa

SEQ ID NO: 14 - protein, 482 aa, Homo sapiens
MGREELFLTFSFSSGFQESNVKTFCSKNILAILGFSSIIAVIALLAVGLTQNKALPENVKYGIVLDAGSSHTSLYIYKWPAEKENDTGVVHQVEECRVKGPGISKFVQKVNEIGIYLTDCMERAREVIPRSQHQETPVYLGATAGMRLLRMESEELADRVLDVVERSLSNYPFDFQGARIITGQEEGAYGWITINYLLGKFSQKTRWFSIVPYETNNQETFGALDLGGASTQVTFVPQNQTIESPDNALQFRLYGKDYNVYTHSFLCYGKDQALWQKLAKDIQVASNEILRDPCFHPGYKKVVNVSDLYKTPCTKRFEMTLPFQQFEIQGIGNYQQCHQSILELFNTSYCPYSQCAFNGIFLPPLQGDFGAFSAFYFVMKFLNLTSEKVSQEKVTEMMKKFCAQPWEEIKTSYAGVKEKYLSEYCFSGTYILSLLLQGYHFTADSWEHIHFIGKSTEPSSWSTHEDGSLHGEYRMNPLCLLQ

SEQ ID NO: 15 - DNA, 1676 bp, Homo sapiens
agactcaacaagagctccagcaaagactttcactgtagcttgacttgacctgagattaactagggaatcttgagaataaagatgagctctgaaaattgtttcgtagcagagaacagctctttgcatccggagagtggacaagaaaatgatgccaccagtccccatttctcaacacgtcatgaagggtccttccaagttcctgtcctgtgtgctgtaatgaatgtggtcttcatcaccattttaatcatagctctcattgccttatcagtgggccaatacaattgtccaggccaatacacattctcaatgccatcagacagccatgtttcttcatgctctgaggactgggttggctaccagaggaaatgctactttatttctactgtgaagaggagctggacttcagcccaaaatgcttgttctgaacatggtgctactcttgctgtcattgattctgaaaaggacatgaactttctaaaacgatacgcaggtagagaggaacactgggttggactgaaaaaggaacctggtcacccatggaagtggtcaaatggcaaagaatttaacaactggttcaacgttacagggtctgacaagtgtgtttttctgaaaaacacagaggtcagcagcatggaatgtgagaagaatttatactggatatgtaacaaaccttacaaataataaggaaacatgttcacttattgactattatagaatggaactcaaggaaatctgtgtcagtggatgctgctctgtggtccgaagtcttccatagagactttgtgaaaaaaaattttatagtgtcttgggaattttcttccaaacagaactatggaaaaaaaggaagaaattccaggaaaatctgcactgtgggcttttattgccatgagctagaagcatcacaggttgaccaataaccatgcccaagaatgagaagaatgactatgcaacctttggatgcactttatattattttgaatccagaaataatgaaataactaggcgtggacttactatttattgctgaatgactaccaacagtgagagcccttcatgcatttgcactattggaaggagttagatgttggtactagatactgaatgtaaacaaaggaattatggctggtaacataggtttttagtctaattgaatcccttaaactcagggagcatttataaatggacaaatgcttatgaaactaagatttgtaatatttctctctttttagagaaatttgccaatttactttgttatttttccccaaaaagaatgggatgatcatgtatttatttttttacttcctcagctgtagacaggtccttttcgatggtacatatttctttgcctttataatcttttatacagtgtcttacagagaaaagacataagcaaagactatgaggaatatttgcaagacatagaatagtgttggaaaatgtgcaatatgtgatgtggcaaatctctattaggaaatattctgtaatcttcagacctagaataatactagtcttataataggtttgtgactttcctaaatcaattctattacgtgcaatacttcaatacttcatttaaaatatttttatgtgcaataaaatgtatttgtttgtattttgtgttcagtacaattataagctgtttttatatatgtgaaataaaagtagaataaacacaa

SEQ ID NO: 16 - protein, 199 aa, Homo sapiens
MSSENCFVAENSSLHPESGQENDATSPHFSTRHEGSFQVPVLCAVMNVVFITILIIALIALSVGQYNCPGQYTFSMPSDSHVSSCSEDWVGYQRKCYFISTVKRSWTSAQNACSEHGATLAVIDSEKDMNFLKRYAGREEHWVGLKKEPGHPWKWSNGKEFNNWFNVTGSDKCVFLKNTEVSSMECEKNLYWICNKPYK

SEQ ID NO: 17 - protein, 9 aa, Homo sapiens
SLLMWITQC

SEQ ID NO: 18 - protein, 14 aa, Homo sapiens
CASSYVGNTGELFF

SEQ ID NO: 19 - protein, 9 aa, Artificial Sequence
  Synthetic
KVPRNQDWL